European Patent Application EP 4 520 345 A1, published March 12, 2025. Title: Product. Applicant: myNEO. Application GB. The sequence listing filed with the application follows.

SEQUENCE LISTING (611 sequences)

SEQ ID NO: 1 - RNA, 2034 nt, synthetic construct
  source 1..2034: mol_type = other RNA
tttttgcgttctctttccctctcccaacatggcggcctcagcaaaaaagaagaataagaaggggaagactatctccctaacagactttctggctgaggatgggggtactggtggaggaagcacctatgtttccaaaccagtcagctgggctgatgaaacgatgacctggaaggagatgtttcgacaacttggcacagtaacaatgacgatgtgtatagggtgcctccaattgaccgttccatccttcccactgctccacgggctgctcgggaacccaatatcgaccggagccgtcttcccaaatcgccaccctacactgcttttctaggaaacctaccctatgatgttacagaagagtcaattaaggaattctttcgaggattaaatatcagtgcagtgcgtttaccacgtgaacccagcaatccagagaggttgaaaggttttggttatgctgaatttgaggacctggattccctgctcagtgccctgagtctcaatgaagagtctctaggtaacaggagaattcgagtggatgttgctgatcaagcacaggataaagacagggatgatcgttcttttggccgtgatagaaatcgggattctgacaaaacagatacggactggagggcttgtcctgctacagacagctttgatgactagaagaggtgatgatagctttggagacaagtatcgggatcgttatgattcagaccggtatcgggatgggtatcgggatggcccacgccgggatatggatggatatggtggccgggatcgctatgatgaccaaggcagcagagactatgatagaggctatgattcccggataggcagtggcagaagagcatttggcagcgggtatcgcagggatgatgactacagaggaggcggggaccgctatgaagactgatatgacagacgggatgatcggtcgtggagctccagagatgattactctcgggatgattataggtgtgatgatagacgtcccccccaaagacccaaactgaatctaaagccttggagtactcttaagcaagatgattcctctgctagtacctcccagtccactcgagctgcttctatctttggaggggcaaagcctgttgacacagctgctagagaaagagaagtagaagaacggctacagaaggaacaagagaagttgcagcgtcagctgagtgagccaaaactagaacgacggcctcgggagagacacccaagctggcgaagtgaagaaactcaggaacgggaacggtcaaggacaggaagtgagtcatcgcagactgggacctccaccacatctggcagaaatgcacgaaggagagagagtaagaagtctctagaaaatgaaacactcaataaggaggaagattgccactctccaacttctaaacctcccaaacctgatcagcccctaaaggtaatgccagcccctccaccaaaggagaatgcttgggtgaagcgaagttctaaccctcctgctcgatctcagagctcagacgcagagcagcaatcccctacaagtggtgggggaaaagtagctccagctcaaccatctgaggaaggaccagcaaggcaagatgaaaataaagtagatgggatgaatgtcccaaaaggccaaactgggaactctagccgtggtccaggagacggagggaacaaagaccactggaaggagtcagataggaaagatggcaaaaaggatcaagactccagatctgcacctgagccaaagaaacctgaggaaaatccagcttccaagttcagttctgcaagcaactatgctgctctctcttgatggtgaagatgaaaatgagggagaagattatgccgaatagacctctacatcctgtgcttttctcctagtttctctccaccctggaacattcgagagcaaatcaaaacctctatccagacaagacaaaataaaactcaccatctcctgaagatctttcttacctttttttaaaaacaaaaaatgaaactattttgcatgctgctgcagcctttaaagtattgaagtaactggag

SEQ ID NO: 2 - RNA, 3929 nt, synthetic construct
  source 1..3929: mol_type = other RNA
ccggtggggtgcagccctgctgaagccccagagctcagcccagtgctgggcacatagtaggcgctcaggaaatgattgctgaatgtggaatgaaagtccccagcaggcaaaaggctgtgacttctgttagtggggtggtggtcctctggggcgagtgtatggagaacttcaaggcctcctcctggctgcccaggaagtagagggcgccaaaggcgacgtgccggccgccagctccaggccgagccccgagcgcctgcaggaacacgccccttcacccggcgcgggacgcagagctgcgagagaatcttgttcagcgcggactcaacgccagggcgccgcctagaggttggtctctgtctcggcctcacccgccgggagaccacagagctgcttccccagccgcccgccgccagaaattggaaaaaaaaaaaaaaaaaaaaaaaaaatccagctggggtctaggaactcggcttctggcacctctgaattctccgagactgtctcctccctccccgcctgtaatgaaccctgtgaagggagacaggccaggaagtcccagaaatatttattcttgtgactctcacaaaatggaaaagggtctcaatttttgtttctttaaggaacttgtgttctgcgtctgtgtctacactgcctcctctcaccaaccaaattgtctagcccccctccagttacgctagaactctgctttatcttcaaggaagaaagggagtggggagaagttacctctaaaccctccagcatggccatcaattttctgaataatttggaggtcaacatgcttttggaaaagtgtttggaaaacgtttgggggtgaaaagaaatgttgcctaactggcctttactcacggagtgaccatcatctcagctagttagtgtatgagcggcaccagcaccccggccatgggtgtctgtgctgagcctctgaaagttgacttatcctttggggagccctcggaaagacacagctggtatctatgggaatggctttggggtgtcctttggcaccatacagataattttgtttttttaattggaatccatggcctgggttcttgggatgggggtagggggaagccacaaagcccctggaaatgtatgcaaaacatatgggtgtgcaggtgcatcatcctaaggctatggcctcttcagtttttccaaagagtctaagactataaaaggtttccatctccttttctcagccagggagccacagagacccaggccagcagtaggctgggagccagcacaccggcccccaccaggtgcccggtaggggatgggtaataacactcttgaatggtctggaaactgctggcccctcagtcctgccgtcctcccagagggaaatcctaatagaagaagtgacagccagtagctgccatctcagtattttgaatgaaaatataacatgataaagagcaaatgagggaggctggaggggcctccccatgcaaatactggaatatgaatgttggccagaaataagatacttcctgccctccagctgttaaagagctccccaattcctcccttttggtgctaggaaggggccagagggcactgcccccagaccaccacccacctctggagagctggggccgagtgggactgcctgcagcagagttaacccttcagaaaattcaaaacctatactgcctagtattttccctgcccgtttattttttaatcagatttttaaaatatccagcagcactttggtgccttttcttggggttggggagtggggttatctatgtgtgtatctatgggaaggtgggtgccttcagtgcactaaaccccctcttgggcctgcagctggacctcactcctgtacctgaacactctgcctgagcctgagctaatcttagccatccattgtgtctcaaaactgttttggaggtgaataactgtgaggcaggatggagaaccttttgctctcccatccagaagggcacctaaccaggcccctggagcagacaaaaggagcaggaagtcaatcacttcgatcccagttctctgaagcccaagaagaaaacggattttccttcgttttggttcggaggcctagtagagaatttggattccaccaagttctcttttttcaaaaaaagtaaacggtccagagcagacaaaaactgtggaaacttgaggcctgggtagtagtggttttgtttgattttgaggctttaaagagataaggagacggtggtggagctccgccacgccgcgtggctctcacttccacgccgaggaagaccgaccggcccctaggtttatcctctgggagcccccggcccaatcagcccccttcaggccttgggagtcaccccgagtcttatcttctgtccccttccagcaagtacccggcaataaacgggcagggctgggcaaaggtctggccgctagaaacggaaaaggaaagagaaaagtaaagttaaacaaaaaacaaaaacaaaaaacccttgggtcgggcgcggtggcttacgcctgtaatcccagcactttgggaggccgaggagggtggatcacgaggtcaggagttcaagatcagcttggccaatattgtgaaaccccgtctctactaaaaatacaaaaattagccgggcgtggtggcgggcgcctgtagttccagctactcgggaggctgaggcaggagaatcgcttgaaccgggaggcggaggttgcagtgagccgagatcgcgccactgcactccagcctgggtgacacagcaggactctgtcaaaaaaaaagaaaaaagaaaaaacccgctttcagcggaaagatgcaaaaaatggaggccaccgggcgtggttgggagagcctgggctttcgcaaggaagcgccagggagcccagttctgctctagcgagaagcagggagcctcatcccaagcccggcgggccgagccgatcatagggtctgcgcggggctctgtggattttccgtgtaggcggcggcttccagtctctgccgggcgcgggctgggtcagcgccgactcctccgagagaagagcgcgcctggcggccggttcggcggaggccaagtcccgggggctggggctgcttctctccacgcggacaaagtgtgcgggcaaagaaaggggccgaggcgggtgcttctgccgctcgtaaatttgtttccccttccttttaatccgcccccggacgtctttcttttcaggacaggaggggatgtaaaccgtttgaagttcatcaacacggtgaagttttattgtatttccggtccccaagatttatacccgggagggggagcgggcggccaggtggactccctcgctacctcggacttccctgccggacacgtggccactcggaccctcgcttctgggcgagggcgggagggagcctggactgggccgcggccgctggctccgcaccttccgacggccgcgcactgccggcaccgccgccgcccaggaactgaccgcaaacgaggccgccagacctacacccgctaccagaccctggagctggagaaagaatttcactacaatcgctacctgacgcggcggcggcgcatcgagatcgcgcacacgctctgcctcacggaaagacagatcaagatttggtttcagaaccggcgcatgaagtggaaaaaggagaacaagaccgcgggcccggggaccaccggccaagacagggctgaagcagaggaggaagaggaagagtgagggatggagaaagggcagaggaagagacatgagaaagggagaggaagagaagcccagctctgggaactgaatcaggaaactcaaatcgaatagggaagtaaaaaaacaaaacaaaaaacaaaaaaaacaaaaaaaaaaccctatttaaatgaaaggagtttaaaaacattttttaaggagggagaaaggagaaattttggtttttcaacactgaa

SEQ ID NO: 3 - RNA, 989 nt, synthetic construct
  source 1..989: mol_type = other RNA
ccaccatgtgaagaaggtccttgcttcctcttcatcatctatcatgattgcaagtttaggcctcctcagccacgtgcaacttttatttcaccctgaagccaaagagaactttctgaaagacaaatttgctcatgctataatagttactgacaaatatttaaaggactaagttgtgtaaggaatctacactgtcaggcagaaccaggattcctggaagtagaactgggctgcttcataagtctgacttcatatgacagctagattcaaaaggatgaaatcagtagaggtgagacctcttgatgccttggcttggaagtcacatattctattggccaaagcaaatcacaaggccaccacaaattcaaggagatgaagaaatagactctacctctcttgattggcttataatatggtcagttcttcagaggaagaggaaaatttcatctggcctcaaatctcagtgatcgcatttgtgggaacataatgtctgaagtaaagactaagtagaagtctgacaagcaaaaaaagaaaaaaagacaaagacactccaagcaagagaaacaacctgagcagaagcacccaggtatgacagaaaacgtagagaggaaaggcttccaaaagcaacagagattcacaggaagctccacagaaaaacgggtggtgcaaaaaattaggcaagagggaaaatggggttaggccatgtaccaacatgttcatcattatacagtgattggacttggaaaggcagaagagaagcaagagccagcatcctcatcttataaacagaaaagctgtctgggcgtggtggctcatgcctgtaatcctagcactttgggaggccaaagcgggcggatcacgagatcaggagatcgagaccatcctggctaacacagtgaaaccccgtctctactaaaaatacaaaaaatattagccgggcatagtggcgggcgcccgtagtcccagctactcgggaggctgaggcaggagaa

SEQ ID NO: 4 - RNA, 4397 nt, synthetic construct
  source 1..4397: mol_type = other RNA
cccccaccccttggctcctgggctgcctggaacctggttggctcaggagctttttatctacagctcctctgtctatgtccccttggcaggtcctttttaacatgagtcctcctccagtgaaggaaagggtcatgccagggcctgcacctagggcctccgttctccagtgggtgtctttgcatgaaacggcctgggccctggcacttgccccaccagcgctgcctgcaaccttgtccctgtacctcgggcctccaccacatccctggacctgcacgaaggagccctgagcatggaagtcaggggaagggaggtctcgacatgagcccagccatggccagagtactgagcccagggccagcagcctcggctggcagtgcagggtgatgggtctgtgggccgggctgcccagggacctcggccctggggtctgaggggcaccaatgccttttgcaggccaccatttccctttccactttccaaatgtgattggacacaggtggatgcacctgcctgcccagcagacagcccggttctgacccgtgtggagctgcgtggactgggctcacctgtgccttcttgcatcaaccaggtgtggaccctgacaaggtgccagccactgtcctccaggagctacctcagggacacgcagggagggactggacagacagatggagcgcagtccttgctgcccggccaagcccttgtgggcagggcagactccttcaagatcatcaaatgaaagcaggcaaaaaccacgtccttttgtgacctaagcttggaagcaatgttgtcacttctgcctcatcctattggttagaagtgagccaggaggtcctgtccacatccaaggtgggagtccccgcaggacggggcctgggaggtgggcccatgggctccagaggggctggaccacagcaagaagaacgaggccaacctccatgggtagcgcagaccggctcaggccctgcccttcccgccggggtcccctgtgacaggacgcaagggcacagctgcggagcagggtgggctgttagagctgggcagaggccacagtggccagagggctggtgagagtggctctcctgctgccctagccactggctgaagatctgcctggggaggagtgggtttgggcggccgggcctaggaccccttcatagctaccactaatactcattctctgctcctgagaaacctcctccaggggcctctggggtcttggagatgagacagagggacctcaggcaggacagacaagagaccctggtctcgggtgtccacagagcgggagccaggcaggctgggcggaagtcctaggcttggaccctgttacgggactttccctgtcagaatgggctcaggagggagtgagtgcgtggtcctcaggtgtgcaagtgccaaggctggagcccaccccctgggaagcagggccagggtggctggggcggacttgatccctggagaggagcgtgggcagccagggcagggaggagggcaggcaggagggaggtccaggcctgtgggccgacagggggtgaggaggcagtctggggacctgagagaaggccgagtggctgtggggtgggtgacctggggccctgactctgccttacccttggccatggggccacattcatgctcggcccccgcccagcctgggctgggaaggcatcagcctggccatgaggcaaggggccggccatgcctggggccagagggggtcccccagcccttcgccttctctccatctcctgagtagggcccctgccctgctctgacagggtggtcaccttgccccgctccgtgcccagtcctgagctggcagtgtctccagcctttgcagcgtggccctgtctgcctctgtgtgtgtctgggctcctctcatttggccgccctgcccgtctacactggtgcccccccacctgcactgtccaccgggccaggctctgtctctgccacctgttgggtgcttgccagactccgccatcctctccgctcccagcttgcggcttctgcctccactggcctgggcctgccctgccgccgcctccttgtgccctggctgtctgctgccccctctgctgcccattggccagccgctgagctccctaccaggaagaaaaagggccaggccatgccggaccaggactgggcacagcctccagcactccaggtggacaggctgagaagcgcggcgagcgaggcagcctgggacgggtgatttctggaacatggggccagccagccttggcgtgaggtgtggacagctgccagcttcttctcagggctgctcacaggcagcgggggagtgaccccgttttctgcttggcacctggcttgccatcccgctctaccccagggcactcagacctcaaactcctcagctgcctggaacaccagggaagcccaggctatgtgagcctgtgcccagcaggccagggggcaccaggacatccccctcttctctgatattccaaaccttcctgcctttgaggaatgcctcccggtccttctggttttctaggccatgggctcaccctggtctgccagctctggagctctgagaatattcctgcaaaatgcacatcccaggcctggccgcagactgtgagtcacaggtagggcctgggatcagcattttcatggattctgcaggcactgctgagagcagctgcccggggtcaagccagggcgtgggctgtcctcatcaggctccccttctcagaggccgcccttctggcctggcctgcacctttccccactcactgcccaccagctgcagacacactcactcctgcctcagggcctctgcacggtgcagacattcctcccacagcttcccagggaggctgaagagcaaggaacctgcctctcctcacggagccctctgctcccgccacacggctggatttttcttggatgccagcgtttgacatctctatgtgagatctgcttcttccctgatcgtgacattccctccaccagcaggcagccgcatgaggaccagcgcctgctcaccgctgtgtccctcctacgtgcggggcaggcacccagcagcaggtgttcggtgcccactgggagcgtgcctgggcccctgctcctgctcctcagagggaacaaacaactgacctgctgatggaggctgtgaacccacacgggttgtctgcagacgtaacggggcatctcctatgacgcttctggagagggcaaggctccacggctgagggctttctttgggtgacaaccatgtgaaatgccatgaccttgtgccaccccgtggcagatgactctctcagaaggtggtgcgtaccctttccccattatggtgtggacacgcagatgtggggcctctcccacctcttacaactggggcaggctgacaaccacagtagaagggacaccctggaactcccagaccacatcataagaggccacgcagcttcctcctggagctctcgggcagctgcccttggagcctgactgccatgctgtgaggaagcccaggtgccaccgaggcggcacatgcagatgtgcagccaatggccctggcagaacctgacaaagtcagcaccagccaccagacctgccagcaaggatgctctgagccgacgtccactccagctgtcgtctgactgcccacgagacaccctgagtgagcactgcccagctaagacccgtcaactccagaactgtgagaggcgatggttccacgacttcctggctgtagtcactgctgttgggcagctgtgggtgaccctgaagggacactctgataagggacatctgcctgcatgtgtgacctgagtcccagcctcagctttctcatgtgaaaaatcaggaccacggtagaccctaccttataaggcagctgcaagagtgaaatacaatggaaaatgtacacaagatagggtggctgttcgacgccctcttggttcttcaaatctaaggcccatgtcaagttttaccatcattttgccatcatgatgagaaaagaaatgagaccagcctgaccaacatggagaaaccccatctctactaaaaatacaaaattagctgggcatggtggcactcgcctgtaatcccagctactggggaggctgaggcaggagaatcactcgaactcaggaggtggaggttgcagtgagccgagatcgcaccattgcactctggcctgggcaacaagaatgaaactctgtctcacaaaaaaaaaaaaaaaaaaaaaaaaagaaatggaacttaaacaaggaaatagtgttttccttgttttgtttcttgcttattgaaagcaccttgcctgatgggttgagggagggattttcataaatcactgttgtatacacacgtagagagaaaataccagcaagtaagggttactgtccccacatttgagtccactt

SEQ ID NO: 5 - RNA, 2442 nt, synthetic construct
  source 1..2442: mol_type = other RNA
cgagactctgtctcaaaaaagaaaagctaaggaccaggtgtttttcagtgacttacccaaggtcacatccttactcaggagcagagtttaggcagtgttccaggtcttctacttctaaatccaacaatgttcagggagctcttcattatctgatccctgtctacctaccactttctatggtgatacccagttcccagccttgctgtcctttttctcctctggcacgtttgtcttcatattttggggcctttgcctacacttatcccacttaaaagcctttccctcacttaaccttctcaaattctgaccaagaactgataacttgcaactcatgattcaagaccttactgaggagtctgctcctttagagtccagtgtgtgtccttctaatactccttgatatggtttggctctgtgtccccatccaaatctcatctcgaattgtaatccccacatgtctagggagagatccagtgggaggtgattggatcatgggggcagtttcccccatgctgttctcatgatagtgagtgaattctcatgagatctggtggttttataaggtgctcttcccccttcaccactcattcttctctctcctgccaccttgtgaaaaaggacgtctttgcttccccttgtgccatgagtgtaagtttcctgaggctttcccagacacatggaactgagtcaattaaattcttttataaattactgagtcttgagtatttctttatggcagtgtgagagcgggctaatacagtccttatcacattttgctactattgtgtttggatttgtctcaccttgtgaacctgagtgagcttcttgagggacaggttcggtgttttgctcatcgttagcacaatacctagcatgcatgcagcagatactcagtaaataatcgtttacatttaaatgaccatgaaaatgggtgaatctcatttagtaactttaaaaagggactatttgttgtacaaataacctgttggctacaaactaaaccaataatatagccaagaaagatgttggctagaattgcagcaagtcatacgtatcgctaaaataaaatccaaagcagcaacctcggagaagaaagacatcatcttggaactactgggcatgcagcaggtaagtggaacatcctctgtaccctccttccctgcagctgtcacagtgagtccatgtttccttgacttttaatcagagccactatccaatgttaacaacacacatacaaaagcagcagctattaatataagcagaagacaagagggttttctacttttctcactaaggaaaccacattttgataattctccaggtggttacaaagaacaaactcaagcaagaatgctggactaaacttagtccaaaaggctaattgtggaatgagatggaaaaaaagaacaaaggtcaatggaagagaattgttgaagtcctaacccccaacatctcagaatgtggctttatttgaagagaggattacctttgcagaggtaatcaagttaaaatgaggtcaatatagtgagtcctaatccagtatggttgatgtcctcatgaaaaggagaaatttgaagacagacacaccaaaggagaatgccatgtggagacacagggagaagttggcaatctacaagccaacgagaatagcctggaacaaattcttccatcacacccctcagaaggaatcaaccctgactgcacctccattgcagagttgtagcctccagaactgtgagacaatacatttctgttgtttaagacgctaagtttacggagtaaatttctgcttgttacagcagccccaggaaactattacactccacctcagcattttcctccaggcatccctcaaccctgttcttccaacatttcccaagaaagaaagaaaaaaatattacttcacatatgtatattataaatcttgccatttcatttgccttcttttaacatcagtgggtaatcttacctcacaaagttagatgtaatatggaaaaacctctacaattttcaaacccataataatcaagttctataatcaccaaaaaagaaaagtacaaaagaaaaccaatggtgagaactcttataaagcaagtacaaagacaaaattggctatgcactatcattaacagaagctatcacggctcctttgtaatcttaagcagctattccatgatcttttctctcgcaatgatgaaccgaacttttgataaaatatttgatctccttttagccaaaactcttctttataagcccatttaatattccagaaggattttctttcgtttgaagaaatataagtttgacattctaaaggcatttgtattttaaagcctacaaaaagatttttggagagtacctggtgaagtaccgacttgcccctgtggctcaaaagttcaattattatagacatttcactcagaacagcatttctgtctttta

SEQ ID NO: 6 - RNA, 269 nt, synthetic construct
  source 1..269: mol_type = other RNA
gagaattatgctgagataggtaacagatgaggatgaaatttgggcttgactgaagtaatgggggctgtctgtgaagccttgcggcagtacagcccagggggcttccaaggcagtcgggcagcatcagtcttcagccgctaagccaagaagatctgggaagcagtcagagagccttgggccagagttccaggggctctgggagtggctgccagtggtctcaaatagtcaagaccccctgctgggaggagcttctatcctgctctgtggaa

SEQ ID NO: 7 - RNA, 1179 nt, synthetic construct
  source 1..1179: mol_type = other RNA
ggggctaggcgtggccgacctcacactctccttgggcaggacctgctgcagctgctctcggggttggaggggaggttcctaggtcaatggagttgtgtacctaggaggattatggctgcctctgctgagtcatgcagattgtcaggaagtgtgagaaagccagcagtcaccggcctcacccagccaccctgccgccattaacagcactaggcaggcagtgcgcagagctgagaacttgccccaggttacccgcctcccagctgctaaacaaaagggaggcttttcagctggttcaaattgttacaaagttcagctagagatttgcttttacctgcggcgttttccccataccactggctgccctcccgaagaattcctgtgatgccaggcaggaatggcctggttggagaccagctagctcccagggcctttcccgctgcttcctctacccctgtatttcgctgggctctctaaatggattcagctccagaggaggaaaaccttgagaccctgagactttcagaaacttattcacagttaccaaagctgaaaatgtttgtggcagggagtgggacatccggcttcagagcaggaactttcattgcaccagtgatgaaaaagagaatgaaatgtgggtgacgttgagaaaggcaagaagatttttgttcagaagtgtgcccagtgcctaaaagggaggcaagcacaagactgggcctaacctccatggtctctttgggctgaagactggtcaggccattggattctcttacaaagatgccagtaagaacaaagagatcacctggggagaggatacagtgatggagcatttgcagaatcccaagaactacatccctggaacaaaaatgatctttgctggcattcagaagaaggcagaaagggcagacttgatagcttatctcaaaaaaagctactcatgagtaataattggccactgccttatttattacaaaacagaaatgtctcatgacttttctatgtgtaccatactttaatagatctcatacaccagaattcagatcatgaatgactgacagaatattttactgggcaatcctgatttaaaactaagactggcttgtggttaaatgaatgtgttcagtttttgaattttaatagtaattccaattcagtaaatgctatcactgtttaccccttcta

SEQ ID NO: 8 - RNA, 4551 nt, synthetic construct
  source 1..4551: mol_type = other RNA
agtcctgcatgcagaccgcagccactgactgttcccgagtcaccaggccactcttctctcctgcctcatcgtcttattcagggtccacgtcattctgccacctatttgaggacaccaggccttggctgtttctgcttcttgtacctcctgagtcaggtggcggtgggggagggcagacgccacacacacctgggtccactggccgcacggctcctggaaatgctagtgtgactttcctaagggttctttcaaaggacacttttagacctgccttttgtcccaaggattctagttgcttcatctttagtaccacagactggtggctaaacaacgaacatttactctgccaggacaacctcgctgccctcgtggttcccagcacccgcccggacctccacaccaggctactgtttccccaaacgagtgagtgtcctactcccttccggcagccctgaccttctcctgcctcggattctttcattctcttctcggctcctaaattcaagctccccttataaagctcagcccagattcccatgataacgtgctctgcgattatttgccgattccatcaacattttttgagtacctgttgtgtgcctgacacctacggcactcagagctggaagtggatccagctgtgagcagaacacagaccctcggggatcccccagcctgctggtagagacgacccccatccagggagatgcgggagcaccgaggagaagccccaaccctggggttcatggatggcttcctggaagaggaagcaaggtgaagtcagaggctaaaaatgcacacatttgcaggtgttgagcaagtagtgtggacgcgtgagcgatgaggcacaatagagcatgaaggcgcgggcggtggcaaagggaacttcgccatctggggaggcatcctctgcccagctttgatcactccctgggatgtgaataggagtttatcttgccagatatatgatcttccaaggtcacaggattttgcgaatttgtatcagatttctcagtttttaaatgttgccaacttgtaactttttaaaatagtcagtggaccatacaagacacaactgtaggccaggtgtgttctgcaggcccttgttgcaacatcttgtctaagtggaattcagccaggcgctgtcatacgcagagcacctgccgagccatgtgacgtgctgctctctgccagccctgatcgccttcctttccagcaggacttgcgcttcacactggaccttgaggccccatggagatctgccattttgggcaggttctgctcacagtgccagtaacttcacctaggagaagagcgacaacttcaaggccgcatgacccatctgattgtcatcacacaggtccccgcaggagaatttccatggcgtttctcactctttgtttgcaaagaatttctttttttatcgttttctttttctttttctattttcttttttcttttttttttgagacagagtctctctctgttgcccaggctggagtgcagtggcatgacctcggctcactgcaacctcggcctcctgggttcaagcaattctcctgcctcagcctcccgagtagctgggattacgggcacacaccacaacgctcagctaatttttgtatttttagaaaagacagggttttaccatgttggccaggctggtctcgatcttctgagctcgtgatccacctgcctcggcctccaaagtgctgggattacaggcgtgagccaccacacccagcctaagaatttcttagaattaatatctgcacttggccccacatcctctgagtgataacttagaactgtcactttaattgttgagagaggatattcagagaatagtgggtgattttacaagcaaggatatgtttggggagcatgttcccggtgcattctcagggtctcgtgcattcttttagacattgaagacatcctgatctccagtggaagcagagccccagtcatacacttatccaccggggacgagttccaagacccccagggaatgcctgaaagctcgggtagtgcttacctctatggatgttgtgcacaaatttatttttccctctttacaacttcatagattgaaggttcgttcttaccaaagatcttagcaaccttagcttatcattccttttatttcctgattaagtggagaactttcaccttttcactaaaaaaaaaaagtgctttacggctgcctttgccacgtgcacatggtcttttgggaccatccttaagtcaaataagggtgacctggatgcaagcactgtgatacagagaaagtccagctcaccaccaagatggctgctgagccgctggtgggcgcggagtgtcgtgtctgcagcgtgaacatgccgggcaaaggaataatgcatgtcagggatagggtggagaaggactgtgccaggcttcatcacactactcagaatggcacacagtttagaacttataaatgatttatttctggagtgatccactgcatattttcagacggtggttgatcgtgggtaactgaaagcaaaacctgactgaaaggggctgctgtgttcatgtcagcaacgctgatgccctcgaggccagaagagtaaccaccaatctggtacctgagcacctggctgtaagtccaccctccatttctggccagggccgaggaattctctctttttctctttattttcctcttgatttgagaaggtcaactctgagcatgctctaaacacaaatcagcatctctacacttcttcggcaccaggtgttgctactgtctttctgattagaaaaaaagaaatatccaggaattctggaagacagtgattgatttgcagctatgctgcaatggagctaagaatcattagcacaacccgtgctggtgttcgacaagatgcccaatcaattcatccgatgacaggtgcgctgtgtctgcgaagcgcgaagccacggagtgaggtgctgaccaggctccaccaggagcaaggaacaagactccccaggggctcctggtccacagaaggcagggacgcccacaaacataccatgagtaaatagttccaatgtgaagaagactgaaaatgccacagaagtgtgagcccactgttttgaaattctttctgctgaagggattgagaagaactcttccataaaggagcatgaccgagccatgagttataatatatacatgcatatagaaagaggatgtgaatacagttgcagaagggcgtcaaagccaaaaacacacagggaatgacttgaggaagctgaggaccaagagcagtgctagccatgccagtgactgtggtcgctgagaactggatgatggatgtttgagtgaccgtcaggaggatcagcatgggaccaggaggatcagcatgggaccaggaggatcagcatgggaccaggaggatcagcatgggaccaggaaacagcaggcgagtgaatgtgaactccactctcaacagggagatgacgtgggtctcggaaacctacagatctgagtgcttgctgtcaggtcatggcagggctctgactgcactgtggagggaacatctgtgtttttgtcctcctggaacctagtgcccctttcctggaggcagcatcctatttgacctgtgtgggtccaaccccacctctctcctgtagcagtggcatgggacccggggctgggccattcgcagcattgccacaggcagcaatggtgattgatctaggagttgatcattgatcctaactgggtgctcaggccaaggggattgattcttggtattttttaatctcttttttccactggaattatagctaatatgatgaagcctagatatactgcgtatctggcttttagacagggcaaacctgcctagaaatgaaaatgaagtcaccacctgtgaaagcagaaacaagagcttgagagagactgagtcctggtgagaatttctgaaccccttgatccagcgatgcctgaagccagaactacttgtaaacttttcagtcatgcaatcctgtcacttctgtttgttcttaagtgcattttgtatggtttctgccgctgaccacggaaacgtccttcactaacagggaagcagagttaccccatttgagagcctcagaaggaagatggcattcatgcaaaggaagcatgcgtttgctctcacttcctgagagaaagcctgaaaatgaagccaatctcattttctttcagagatgagtctcttgatcagagaatgcctcagttccctgtatctgaattttagcaagcgagagaatgcatttaggacaagcaacagcgatggctcccgtgtgttcttggctgctctgtttctaaatgaagattcacctggaggcagcctttgctgcagggacacccagatctcaccttgttcttgttcttttcaatcattttagcaaaggctcagcctactgatccgatttagagatgagccatgaaagcagatatttagataatattttcccaactgcctggagcattaggttagaactagtgagataaaaatataatgaaaataatagaaagctttgaccctcagattt

SEQ ID NO: 9 - RNA, 277 nt, synthetic construct
  source 1..277: mol_type = other RNA
aaccaggataagttgatcaccctccctgagagtttgggattctatgaggactcctgtctagagtgcagcgccactgcgagggtggtcctttattgtcagaaacctcattcccagaaggagacatgcagtggaaactgagcgtcctctgccctgcggtgcccagctccattcaagaaagcacacctgtggatgagaggcgcaattaacgttatcagtcgtgaaggatcagaaggaaaacccagtggccgttgggaatttagagatggtgtttcgccat

SEQ ID NO: 10 - RNA, 522 nt, synthetic construct
  source 1..522: mol_type = other RNA
agaggtaggaaggctaaactgaggaattatgtctgacagaagggaagaagaaggtaatgtggagtgggtagcctccatactgattaagaagggtacagacttaccctccactgtgagaattacctaaagctcggtgtctgtgatggtctacagggcttccgaggcgatcaggcagtggcagtcttcagctgcaaagccgagaagatctgggaaggagtcagtcagggagccttgggccagagttccaggggctctaggagtggctgccaggtgagttgaacagtccgatttctagtggggtcctgcacagatgggacacggcttaggaggaatcctgggctgcgggcattccttggcctggtggccagatttctggcacttgtagcaagctcctgggggaggtggttccggaggaacgcctggccactgcggtttaggcatttggaagttcttgtgtgctggagatgtggctggggtttgtctcacagtggaggcaaggaattgcaactcaaaaatatgttg

SEQ ID NO: 11 - RNA, 398 nt, synthetic construct
  source 1..398: mol_type = other RNA
gcagcagctgctgcacagagacatgatggctaggctaaaaacagtaaggtcaagttgtttggacagaaaggctacagggtgcagtcctggctcttgtgtaagaattctgactgcactaaccatgcctaggaagggaaggagttgttgttttataagggattgaggtttgggagattgatcggacacgatcagcagggaaagcatgtgtgtttgtatgagaattatgccgagataggttttagaagcccatgctgtagcaggcaagtgataacaggctttaatcctttaaagcgtgctgtgggatgggatattggcgttgagcagggtaagggtgattaggttttaatcggatggtaatgggcatgtgatcggttgccagggaagtagagatgtcccat

SEQ ID NO: 12 - RNA, 1865 nt, synthetic construct
  source 1..1865: mol_type = other RNA
tcctcagtgtactccatatctccggttggcttcacaattactcagtattactaaaccctggtgcaaggcacaatgctgggccctggagagggcctgaaggagcataagataacaaacattcctgccctcaaggtgcttactaacggagcccttcagatactgtagatatgtactagagaactctaccttgagaatttataataagtgctaaataagatatacagtgagtttctatgggagtttacaatgagaaagaacagcagtgtggagaagagtgatcagggaaacttcattctgtgaaaaacaaaaagtttcagtcctttgtttaaaatttgcttttctttcatgtttctcatccattttcttttgcctttttcattaaattgctactttcgctaagcaatattgagtattctaggcacttagtaaacgggatcattaaacctcttttagaatttagctgaggagctagaatttgagtatgctggtatcaaaggatggtgcaggaaaaccaagtacaactgattgtaagcatcttaatttcagaagacccttttctgattactatttctaaagatgttcatatagttttaaggctactgttactgaaacagtgtagattaggccacaggttttaagtagcaggtgaaataaaatcctacactcactggtattcaaggtgagcatcgaagttgcaggttttactctttacaccagaatcccaagtgtaaagcagctagactcttttgctctagaaaacaatatcttaacatttgcctcactttcttcaactaaagaaaaatgatagggccacgtgacattcttctagaaaattttttttaaaaaaaggatctaccttatataacttgactggggcccttataacttattagttagaaagctctgatctcatgccttctgttttctttgttttgtattccattttgctcagctttcggggcaccatttcattccctttacatattctggatttggggtttgtctcgttcccaccttccacattttctttgctgattctgaatgtagctttggaggagcatggataaaataaaagagtgcagagcttgaggatgaggacatgctgccctgcaccccgtcatgtgctctgcttctgatttaccaactgcagagataagcagtgtatcctttctttcatctaagacgagtaatactttcttccatggaaaaagcagtagttcaatcttaaaaagaaattaggtcctttagaagaattgaagcactaaagcaaactaaatcaagttttgttaccattttgtccagcattgttgtttgttcaatggtacacaggacagtagttatttgaaagcatgtgttagatcatatttatgtagtagaattgtagaaatacagaatttataagatacaagaaagctttgaagcttctgcagatgtttcagatccactcaattcaatgccctggttaatactgaagtgatatgtaaatttaatattatggggaaataatggaagaagcccctgttcttctacctgaacatggagtctatcttttgggaaatgaccagttttgcatattggcctcccactctggtggttttcattctacatgtagtaaggaaactgcctagaattgttttggtccctgttgatcaacggttagcaaattttagcatatatcagaatcagtttcagaaggcttgtcactcaaactccaattcctatttcaaactacctttaagatttaaatgttcatctctcatttagtatatcaagactgacttaaattttccctactctagcttttttctaatttccccattttgttaatgcaacatcttttttccaattctccaagtttagaactt

SEQ ID NO: 13 - RNA, 830 nt, synthetic construct
  source 1..830: mol_type = other RNA
cagcccgcctgcacccaggtgaaatagacagccatgttgctcacacaaagcctgtttgctggtctcttcacactgactcgagtgaaatttggtgccgtgactaggatcgggggacctcccttgggagatcaatcccccgtcctcctacactttgctctgtgagaaagatccacctacaacctcaggtcctcagaccaaccagcccaagaaacatctcaccaatttcaaatccgtgatagatcacaacaagagatcatgaagagggcatggccgccatgtcattctggagagagacagagtaaaacaaagaagacagagtcttgttctgcaacccaggctggagtggagggcagtggtgtgatctcggctcacttcaacctccgcctcttaggttcaagtgattctcctgcctcagcctcccgagtagctgggactacagcagcctctctacaagtctcctaacttaacctgatgggaaaacacttcctaccactaacagcatctacttgattactgatactttgatcatggagtttgggcatgccacttgatagaaatttgaagagcaattatatttttcaaaaagagttttgaataatgttaagatagattgcaacatgactatcaattcttcccttcccatcaaaggagagagtccgtttatccagcctttgaatcttgattattcatgtgacttgcttcacccaatgtaacattaataagcacaatacaagcagaggcttgccaagaacttggtttgtttctaatgcttagaagaagaatggtgtatgccatatttctgcatttagaactcacgtggagacatgtgt

SEQ ID NO: 14 - RNA, 1572 nt, synthetic construct
  source 1..1572: mol_type = other RNA
caccagtggcctcaggttactgtgtgtacaaggtgtttgtgggatatttctggtctcccacaatttcagctgatgtccagagttaaagggctctaagtaagtaccccaccttctataaagtgttgctaaggaaagccctcaatgctaaggctttgatacaaaataccattgatccaccttcccctcaatctttttgttttgttttgttttgtttttgagatggagtctcactctgtcgccaggctggaatgcagtggcgcgatctttgctcactgcaacctccgcctcctggattcaagtgattctcctgcctcagtctcctgagtagctgggattacaggcatgccccaccaagcccagctaatttctgtatatttagtggagatggggtttcaccatgttggccaggctggtctcaatctcctgacctcatgatccgcccacctcggtctcccaaagtactgggattgcaggtgtgagccaccgtgcctggcccccctccatctttttgcatcagaagagacatgaaaagggagaaaatggtagttgtggtcaactgtgtggtcagcagtgtttacagtggcagactgtctacagaggtgaagaggggtgccttctcttctccctttgcagaggccaagtggggaaggttgaggagcaagaaagggagaccagcatttccatttcccagttgggttcccatttgggcacctgcctgtcgggccatctgcccggtaggaagcacttcctcgataaccgtgcagcagtgcctgaccccaattcatgcggctcaactgtggatttctctctttagtatgaggggtacttagcagagttggttttttttttttttttttttttttttttttttcagatttggcctttaactggcaaattctgggtcaggaagagcgcccctcaacattttttgatgctaatccttcccccccaaatctgccactggttacagtaactcagctttcccacttgagcagtttgagggatgcagggtctgacaggagcccagaggccgttcagaggatgggcaccaacagtaccctggctccaaacagggcagccaggtgcaaggtgggcacagggcttagcagggaaggtgggccggcaaggccaggtgcatggcaggagtggcggggagcctggtgggctgtggggagtagaggtagttcatggccagcctggagctgagaacatggagaaagaaccccaaactcttaatttttctgtagaacttggctggtgctcagggctgctggcagcctcagctggaaatctgtttacccagagaacgaagcatcagataagctttgtggtggaagagagccatgattctcagtctaaatgttgaaattagagggagaggcaaagagaatccaatggaacttgtggccggtgaagctctagtgagcctgaggcagtgacttgggtctaaggtgaagccttatttatggagaagcgatcccaggcgaaaacagctgttggccagagttttggagaaacatgagttgactcagaattaggccatgaacttaggttattatttgccttttttcc

SEQ ID NO: 15 - RNA, 12606 nt, synthetic construct
  source 1..12606: mol_type = other RNA
gctggtaatggtcacactaggtggcgtccgcgtgaggtggaggtgtcagcggctcctgtctgcagcttcctggggtcctggcggcgctcttctcctgagccagaatccagcaggaaggacagaatgggcgctagagtgtgaaaagagggcgaactcacgtggatgtgactctccgggtcgctcttccctgtcacccagctcctcctgccggtttcctgtgggcatcgcctgcattgcttttatcccggggacggattaggggggtccagaggaggacttgctggcacaaataacccaatggaggctttcgagcacggctggctggggtttgcgatccaacggccttttgctgacctgaaagtcaacgcaaagctcatcttcattctagagaaaaagaagcctcatatctgagatcaggaccccgctttctccttgacattccacagcaaaacgtgaacagctgaacaaacacacagtccggtttcccgagaccaaagggtcaggggaaacccccgctgaaaacgtgcatcagtggaacaactactctcttccaggtcccaccgagggcaaagaggagaaatagaatccctcacaagaaatccacaacttctagaaatccgcagcacacacagaacacacttacctctcacagctctacggacacttcacaccccacagtgggaccgtctgattgcatttgcattttgggacatgtagtccagaaagcttaaatgatgcgagaaaaaccacaagtcccacaatcctccgcgtctcgcaattgacagccccagatcatccaggaacgccccctgtcggctctttctggtcagaggttcccccgttaatataaaagcttttaatcatggatttttttctttgttttcaatttctgtgggcacttagtaggtgtatatatttatagtgtacataagattttttttcttttttcttttttttttttaagacggagttgttgttttttttttttgaaaaaactccagtctggagtgcagtggcacgatctcggctcactgcaacctccctctcccgggttcaaccgattctcctgcctcagcctcccgagtagctgggattatttttgtatttttagtagagacgggggtttcgccatgttggccaggctcgtcttgaactcctaacctcaggtgatccgcacgccttgacctcccaaagtgctgggattataggcgtgagccactgcgcccggccatcttttctcttattttttgtctttttttcttttctctgtgcctgtctatgctttacccacatgagatgttttgatacaaacatgcaatgtgaaatgagcacgtcattaatcatggatctagatttgacttttttttaaagtttttgtatttttagtagagacagagtttcaccatgttggccaggctggtctcgaactcccgacctcaggtgatccgccaacctcggccccccaaaatgctgggattacaggcctgagccactgttcccggcctagatttgactcattctaaacatcagagtttgtgatccttttcattcacaacgacagtatcaagttatttgctattggtaaaataccttgaacttgtgaagaaatgtgtttatacatatctgaaaaagtgatagtttgttgttgttgttgttgttgtttgtttgtttgtttttgagacggagtctcgctctgttgcccaggctggagtgcaatggtgccatttcggctcactgcaacctccgcctcccgggttcaagcaattctcctgcctcagcctcctgagtagcagggattatgggcgcatgccactacgcccggttaatttttttatttttagtagagacaaggtttcaccatgttagccaggatggtcttgatctcctgacctcgtgatctgcccaccctagcctcccaaagtactgggattacaggcgtaagccactgtgcccagccaaaagtgatgtttttacagttaatatgaagccaaatatattatacctggactaatgtacttaacctgcttggcttctccaattttatttatcatattttttttattaagttaatcaaacaaggcctgcgtctcactcccagggattctgatctacaaatttcctaattgttcctaatgtgtagacaaccagaactgccgctctgcagcatcacctaaatcaataaatgtataagtgtctttggacataaaggtgggcggccagcagggaccttgaagaccacctaaggactcccttcccccattttaagatgaattgggctgagtgcagtggttcccacctgtaataccaacactttgggaggccaaggcaggaggatcacttgagcccaaaagttcaagaccagcttgggcaacatagtgagacccactcactacaaaaaataaacaaaattagcggggtgtggtggtgtgtgcctgtagtcccagctactcaagaggctcaggtgggaggatcactttgagcccaggagatcgaggctgcagtgagccataattgtgcgactgcacttcagcctgggtgacaaagtgagatcccatctcttcaaaaaataataataataaataaagatgaactgaagtgcagagaagtaatgtggaagcttgagaaagagtttttaggtttttggttctatcattgtatctttggaggtaatattggcaaaatgaccatttagtagtttgcccatttctgctttttttttttcttttttttgagacagggtctcgttctgtcacccaggctggagtgcagttgtgacatcacagctcactgcagtttctacttcccaggcccaagggatcctccaacctcatcctctcgagtagctgagatcacaggcatccaccaccacgcccagctaaattttgttattttttatttttgtcgagacacggtctcactatgttgctcaggctggtctcaaactcctgaactcaaggaaagctcttgctttggcctcccaaagtgctgggattacaggtgtgagccaccatgccgggcctgcttatttcgacttggcagcatcgtttcatgaagcccctgactctgtgacaacatacagctctccagaaagatgctttgaagacaaaacagaatagagcacacagccctccatgtctcttccaagtcactatattcattaaaagataaatgactctggtcattgccttttcctgcacaagataatgtctgatggggttagtgatgatacctctgtaatccataaccagatatactcttgcacccaaactttgatatgattgtgctttaatgtaactttgaagcaagtttaatgtgattttgcaggcgccgtacactcaccacttgtatatgagtggctgaaattctgtgttggaccagtctgatggaactgctcccacactatagccctcggtctgtaatcctcagtaagacttgtaagtaaaactaactttaattttttttttttttttttgagagagtctagctctgttgcccaggctggagtgcagtggcgcgatcttcactcactgaagcctctgccttcccggctgaagtgattctgctgcctcggcctccggagtagctaggattacaggcgctcgccactgcgcccggctaatttttgtatttttagtagagatggggtttcgtcatgttggccaggctggttttgaactcgtgacctcaggtgacccacctgcctcagtctcctaaaatgctaggattacaggagtgagccactgcaccccgccacttttattattattattattgtatttatttatttatttatttatttttgagacggagtctcgctctgtcgcccaggctggagtgtagtggagagatctcggcccactacaagctccgcctcccgggttcacgcgattctcctgcctcagcctccggactacaggcgcccgccaccacacccggctaattttttgtattttttttttagtagagacggggtttcaccgtgttagccaggatggtctctatctcttgacctcgtgatccgcccgcctcagcctcccaaagtactgggattacaggcgtgagccaccgcgcccggctatttatttatttatttatttatttatttatttattttttgagacggaatattgctctgtgcccaggctggagtgcagtggcacgatctcagatcactgcaacctccgcctcccgggttcaagtgattctcctgcctcagcctcccgagtagctgggattacgggtgcccgccaccatgcccggctaatttttgtatttttagtagagacggggtttcaccatgcttgtcagcatggtctcgaactcctgacctcgcgatccgcccgcctcagcctcccaaagtgctggaattacaggcatgagccactgcgccctgccactttaattatttaaaagcttatttttttattttggggacatggtctcactctttcacccaggcgggagttcagaggcacgatcactgcgcactacagcctcaacctcttggactcaaaccatcctcccacctcagcctcctgagtagctgggactacaggtgggccaccaagcccagctaatttttgtatttttttgtagagacggggtttcaccatgttgcccaggctggtctcgaactcctgggctctaggctttccaaagtgttgtgattacgggcgtgagctactgcgcctggccgattctttttaacttagtacacagggagtagtagctccagcaacagcgaaagtcagtagctgtaggatctactaggcggggaaactcatatgacagccccctccttttttttttttttttttttttttttgagatggagtttcactcttgttgaccaggctggagtgcaatggcgccatcttggctcaccgcaacctccgcctcccgggttcaagtgattctcctgcctcagcctccccagtatctgggattacaggtgtgagccactgcgcccggccaccccctttttttttcaaggctgcagtgagccatgatcctgtgactgcactccagccactgacagccctttctgcattagttaacctgaccacatctgctgaaagaaagcaccagaagctagactgaaattttcgttgtcaaaaaaattataatcccccccaaaatttaaaaattataatccagcacattttctgcacacattttctgggtatttgatcataacttttaaaaatgtgagaacagtgacattctccttccccattcaccaattttactatgaaaaagttcaaacctaggttattttttcagttctccaagtggaatgatcatcactaatagagattggttgggaattctattgtgcttctaggcccccaaaaatctcatgctctgaggaaaagttagctgagttttcaatttttctcatagtgctggaaaatcatccctggacggtgaagtcatccaagtcttttttgttttgttttgttttttctttctttctttctttcttttttaatttttgtatgctttgtttctatttctttttttttttgtcatccaagtcagctggtgaaacacacaatttcacttgatagctactgagagagtgtaatgggccacccattctagaattctcaagggctaggaagttcctttgataccctcatgggattaggattagggctttagtctttttctctctctctttttttttttttttttttttttttgattacaggcgtgagccaccacaccaagccccattatttatttattttattttatgtatgtatgtatgtatgtatgtatgtatttatttattttgagacggagtctcgctctatcgcccaggctggagtgcagtggcgcaatctaggctcactgcaacctccgcctaccgggttcaagtgattctcctatgtcagcctcccaagtagctgggattataggcgcccgccaccatgcccagctaatttttgtatttttagtagagacgaggtttcaccatcttggccaggctggtcttgaactcctgaccttgtgatccacccgcctcggcctcccaaagtgctgggattacaggcgtgagccaccgtgcctggcctagtgtttttctcacaactccaccccatccagaattaatgactaaatccttgactggatgatcaaagtaaaagaatctaaattcaccacattgctagtcttttctttttatccaggctgtgaattaaataagaaatctgctgcagtggctcatgcctgtaatccctccccttggggaggccgaggcgggcggatcacttgagcccaggagctggagaccagcatgggcaacatggtgaaaccctgtatctacaaaaaatacagaaaaattagctgggcatggtggtgtgtgcctgtagtcccagctacctgggaggctgaggtgggaagatcgcttgagcccaggagatttaggctgcactgagccgtgattgcacccctgcgctccaacctaagcgactgagaacatgtctcaaaaaaaaaaaaacaaaaaaaaaaacacaaaacaagttagaaataatcacataacacatcagcatcaaacaggccttttaaaatgtcgtttttgaccatcctggctaacacggtgaaaccccatctctactaaaaatagaaaaaattagccggccgtggtggcgggcgcctgtagtcccagctactcgggaggctgaggcaggagaatggcgtgaacccggaaggcggagctcgcagtgagccgagattgcgccactgcactccagcctgggcgacagagcgagactccgtctcaaaaaaaaaaaatgtcatttttgtatatggatgatgagtacatgaatgttcactgaggaattctttgaacttttcgtgtttacaattttttatgataaaatgttgggggaaatgttactttctttttttttttttttttttttttttttgagacggagtctcgctttgtcacccaggctggattacagtggcatgatctcagctcatggcaacctctacctcccaggttcaagcgatcctcctgcctcagcccccctagtagctgggattacaggcaagcgccaccacgccccgttaatttttgtattttgtatttttgtaattttgtatttttgtattttgtatttacagggatgtcgccatgttaccaggctgatcttgaactcctgacctcaggtgatccacctgccttggcctcccaaagcgttgggattacacgctcgagccaccacacctagaccagatgtaggtttctaatagctttctacatcctgaaggaaaacaggcagtgagggtgaaagttgcttcaaattttagaaactgtgaacattctgtggaaataaatccttattatttgagcctctttttgaattaaggtgtccaaacccttttgaattaacatatgatccagcaattttacttctaggtatgtacaccaaagaatagaaaacaggggccaggcgcggtggctcacacctgtaatcccagcactttgggaggccgaggcaggcagatcacttgaggtcaggagttcaagaccagcctgaccaacatggagaaaccccgtctctactaaaaaaaaaaaaaaaaaaaaaattatctatatatatatttatacatatatatatataaaattagccaggcatggtggcgcatacctgtcatcccagctacttgggaggctgaggcaggagaatcacctgaacccaggaggcagaggttgtggtgagctgagattgcgcctttgcagtccagactgcgcaacaagagcgaaactcagtctcaaaaaaaaaaaaaaggaaaacagaaacttaagctgatatttgcacaccaatagcagcattattcccatagacaaaaggtggaaaccagcaatgaccatctaaaaataaatggataggccgggcgccgtggctcagcactttgggaggctgaggcaggaggatcacttgaggtcaggagcttgagaccagcctggccaacatggtgaaaccctgtctctactaaaaatacaaaaattagccaggattggtggcacgcacctgtaatcccagttagttactcgggaggctgagacaggagaactgcttgaaccccagaggcggaggttgcatgggctgagattgagtctatgtactccagcttgggcaacagagcgagactccccctcaaaaaaaaaaaaaaaaaggataaacagttggtccgggcggcagctcatgcctatagtcccagcactttgggaggccaagatgggaggatcacttgggcccaggagttcgagaccagcctgggcaacatggtgagatcctgtctgtacgaaaaatacagaaagtatccagctgaagtgggaggaggatcacttgaggcctggaagcagaggttgaagtgagctgagatcgcgccactgcattccagcctgggcgacagagccaaaagctgtctcaaaaaagaatgaatgggaccgggcgcggtggctcacggctgtaatcccagcactttgggaaaccaaggcgggtggatcacctgaggccaggagttcaagaccagcctgaccaacatggtgaaaccccgtgtctactaaaaataatcccagctcctcgggaggctgaggcaggagaatcgcttgaacctgggaggcggaggttgatctcgccattgcgctccagcctgggcaacaaaagcaaaacttcgtctcaaaaaaaaaaatagacaagaataaatgggctgggtgaagtggctcacacctgtaattccagcactttgggaggccgaggcaggcagatcacgtgaggtcaggagtttgagaccagcctggccaacatggtgaaatcctgtctctactaaaaatacaaagagtggtggcatgcatctgtaatcccagctacttgagagatggaggcaggagaatcgcttgaatccgggaggcagtggttgcaatgagccgagatcatgccactgcactccagcctgggcaacaagagcaaaaactccatctcaaaaaaaaaaaaagataacatctcatacagtgaaatattattcagccataaaattaatgaattcctgatatatactacaacatggatgaaccttaaaaacattattctgaatgaaataagactgacctcaaggacaaatattgtatgattccatttatatatatataaagtactcacaaagtcatagagatagaaagtagaaaagaggttgccacgggggctggaggagaagggaacagggagtaagggtttaatgggtacagagtctcagtttccacccttgggcatgaaagataaagttctggaggtaagtagtgatgatggttacacaacaatgtgaacatattctatgccagtgaatttacacttaaggttaaaatggtaaattttatgtatactttggcataatttaaaaaaaagtttgaaaaagaaaaaagacaaaacaataatcgtctttggagaagtctgttacactgaatctggagccaagtgaacagaaccctgattttgatcccttttctctcaaaagcccttcgcagtctctgaattaagtctattagcatgttcctcccatagtgctttgcttcatatcaacaaaaacctagctaagtgaaatcagcaacgatatgcagaaaccacctacgcaggtcacaaacatctttctatgattgtataattttcaagcaagcaataagtgaagatttttccataggccctaaactcacctttgcgaaataggaagctggtttattgggagtgatgagcagggggcgtaacaaattagctttgcgcagtggcagtatcgtagccaatgaggtctatccgaggcgcgattattgctaattgaaaacttttcccaataccccgccgtgacgacttgcaatatagtcggcactggcaatttttgacagtctctacggagactgaattttcttgcagttgaacaacagaggctttttttgtgtgtgtgggggtgcttggttttgggaggttgaagagtacttgttcgcaaactctctaaatgagagatggggaagtgtcttaccagctgattcgcgagagcacctgcaagtttacctgttttagtgatttgcgtttatgaaagttggagttgctgattttgtgatctctacttttaaggtaaaagcagggcggtgttgacttttcttgccagttggctgtcctgttttctttctcgcactgttttctttttgagacgaagtctgtcgctcaggctggagtgcactggcgtgatctcggctcgctgcaaactttgccgaacccctgtttagcgatttccgtttgtgaaagttggagttgctgattttgtgatctctacttttaaggtaaatgcagggcggtgttgacttttcttgccagctggctgtcctgttttctttctctcgcactgttgttttctttttgagacgaagtctgtcgctcaggctggagtgcactggcgcgatctcggctcgctgcaaactgccgcccgggttcaagcgattctcgtgcctcagcctcccgactagctgggattacaggcgcctgcccaccgcaccccgctgatttttttgtatttttagtagcgaccccgtttcaccatcttgtccaggctggtcttgaactcctgacctcgtgatccacccgcctcggcctcccagagtgctgggattacaggcgtgagccaccgcgcccagccgtgttctccattcagattttgtcacagtgacgtcctaaaattattcccaactccccccaccctgctgtttccgcaccctcgagcacagctagtcgtccgtctgcgccctccaggctcgctttcccactgctcactctcctcgctcaaaattcaagtctcaaccgagtcatctctgtgacgtcacgttgatttgcataagattccccagcgtcccaagcgaatattcttatggttttcaaaacctgaatgtttgacacgggatgttccaacaacaagaaacctcctatgcagatgggccttaaatacggctggtggagtgggaacacgtcgtatacacggacacacgggcaggcactcaccctcaatgtaatggtagtcatcatccgtgggggagcggggcgcgaacagaacctttccagctttgcgcagtggcagtatcgtagccaatgaggtttatccgaggcgcgattattgctaattgaaaacttttcccaataccccgccatgacgacttgaaatatagtcggcattggcaatttttgacagtctctacggagactgaatttttaaaagtctaaagaaaagggttttaggaagttgtattatagcaggttgtgtcttatgtttggtttgataagttatgagctgttcctatgatagttttttggttgttgttcaggagtattccgtgattgaatgtccggggttctgtgcgggtactgtgagttgttttccaaaatgtatgacactatgttgggaactgggttctaactaagacagttatcgttaatcttttttatccaaatgcagccagcgagtgagctactccacttcctttgtcactgaaggtcacagattcccttaaagggaaggggaactctaaaactaacacattaatacatccaaagtcttcctttttttttttttttttttttttgagacggagttttcgctgtttcccaggctggggtacagtggcgcgatctcggctgactgcaacctccacattccgggttcaagcgattctctgtctcagcctccggagtagctgggattacgggagcccaacatcacgcccggctcatttttgtatttttagtggagacggggtttcgccttcttggccaggctggtttcaaactcctgacctcaggtgatccgcctacctcggccttccgaagtgctgggattacaggtgtgaaccaccgcgttttcttccttttaaagcgaccaagagggaaaaaggcacagaagattgctcaggtcctactgtggagtcctcggcagagctggggcttatcaggttctcttgcccctagtgtggtacttgttcccactacaccagcctcttccagtcttacctttttacgaagacctgggctgtccatggacagaggtcctcaggagtcacaactctgggcatggcggatccagctggacctgcttaggacaccgcccataaaagactcctccagcctgtagcaaaaagaggtggcaaaaagggtggcaacagtacctacaaggtcaaagacggtgctgggaaaaacagctccagtggcaaattaaactcagtccccagttcaaggacctcacagactggagacgtggaggcgaaggtagcagtgagctgaaattgcgccactgcactccagcctgggtgacagtgagactctgtctcaaaaaaaaagaaaaaagaaagaagaagaagccgggagcggtggcccacgcctgtcatcccagcactttgggaggccagggcgggcagatcacgaggtcaggagttcaagaccagcctggccaacatggtgaaaccctatctctactaaaaatacaaaaaaaaaaaaaaaaaaaaaaaattagccagccatggtcgtgggcgcctgtaatcccagctactcgggaggc

SEQ ID NO: 16 - RNA, 441 nt, synthetic construct
  source 1..441: mol_type = other RNA
gagtgttttccaggacatgctagttccaaaagatactccttaaaaaagagttcgatagtcaaaacgttgcttccagaagaagactgtctcattactgttacatctctggccctggagtagcccctggcaaatatgtactcagtacatgtttgcgagacgcatggacttgtagaacagttccacagctgtccatcactgatgttccatacctagcgatgcggcccctcgaaacgcactggagagctgggcagaccaaggataatttcacagactttaggagacttgccctcatatctcataatcttcgctcacaggacgctggacattcaaagaaagaaaaagaagtatagaaaagagagaaaaacgtcaagaactccagcataaagtcctcttaataacgcgtctttttataatcatcgggcaataaatttctgaatggac

SEQ ID NO: 17 - RNA, 2490 nt, synthetic construct
  source 1..2490: mol_type = other RNA
acgtggtggcgatattgagctgtgtatacctacagccgctgagagccggtattccaacgccatgagacgccttctgtcgtgagcagttgacaagaaagacccagcacttactgcaaccggaaggagcggttcctccctcgctcgcgcagccgctcttccccgccactccctcggtgcccgccagcacattcccagcaagccctgagtatatttgcatatcaactcactacatttttttcttctaactaaaaaatcgaaaggacaaattccagattctccttgtgaagtcttcctttcagttcagaagaaatggaattcgctcttcaacttcaggaagttgaaataaagagttgcttggattttgtgttcacctttaccaaaaaatggatttggtaacactgccaccctgctttggtgacagagaaagcaaaaagggcttctgtcgtgagtggcacacgtagggcaactcgattgctctgcgtgcggaatcgacatcaagagatttcggaagcataattttttggtatttgggcagctggtgatcgttggtcccggcgccctttctttactgttatatgttaggcgaaatattacgcgtttggagtaagtggtgctttttgtaactgaaaagagattctgtgtgtgtttttttttttttttagaggctgcatagttatttgtatgaaccgcaggtgacctaattagcaaggtaattcagacctgtatcctagcacttaagaagtggaagtgggataaccctgcgtgttctcgtgtgggaggctagcttaagcaacaaagcaggaaggccccaccaacaaaagaatttaaaaattatacgtgcgtggtggcgcgcgtatgaggaaattatttggcaactgtgttacagtatagcagcaaatggaatagacctagtccctgactttaggagacctgcctcagccccccgaatggctgggactacaggcgtgcgcctccgcgcccagctaatttttgcatttttggtagagacgggttcaccatgttggccaggatggtctccatctcttcatctggtgatccgcccacctcggcctctaggagtgctaggattacaggcgtggccatcgcgcccggcctgcaatgttattttatgaagcagaggaaattgaaattaccttcaccaggccttagcaaactttttctataccttataccatacacaaaagattaattcaaggccgggcgcagtggctcacgcctgtaatcccagcactcctagaggccgaggtgggcggatcacctgaagtcgggatttcaagaccagcctgaccaacatggagaaaccccttctctaactaaaaatacaaaattagccaggcgtggtggagtatgcctgtaatcccagttactcaggaggctgaggcaggagaattgcttgaacccaggaggcggaggttgcagtgagccgagaccgcaccattgcactccagcctgggcaacaagagcaaaactccgtctcaaaaaaaaaaaaaaaaaaaagattaaagacctaaatgtaagaccttaaactataaaactcttagagaaaacacaggggaaaatgacatcgaatttgtcagtgatttcttggatataaacaatggtttacaagcaacaaaaaataaattggtcctcatcaaattttaaaatgttaacattaattttaaaattaaaatgaaaaacccggccgcgtgcggtggctcacgcctgtaatcccagcactttgggaggccgaggtgggcggatcacctgaggtcaggggttggagaccagcctagccaacatggtgaaaccccgtcgctcctaaaaatacaaaaattagccaggcctggtgtcaggcgcttgtaatcccagctacttgggaggctgaggcaggagaattgcttgcaccgggaggcggtgttgctgtgagccgagatcgtgctactgcactccagcctgggcaacagagtgagactctgtctcaaaaaaaaaaaaaaaaaaatagccgggcatggtggctcccagcactttgggaggctgaggtgggcagatcatgaggtcagaaggtcaggaccaacctggacaatatggtgaaaccctgtctctactaaaaatacaaaaaatttagccgggcatggtggtgcatgcctgtaatcccagctactcgggaggctgaggcaggagaatcgcttgcatccaggaggcagaggttgcagtgagccgagatagcgtcattgcactccagcctggacaagagcgaaactccgtctcagaaaaaaaaaaaaaagaaagaaagaaaacccttgtacatcaaaggacactatcaacagagtggaaagacaatccacagaatcagagaacatatttgtaaataatatatctgataagggattaatatccataatacataaggaactcataactcaacaacaacaacacaaacccagcccagttcaataatgggcaaaaggacctgtatagacatttctc

SEQ ID NO: 18 - RNA, 221 nt, synthetic construct
  source 1..221: mol_type = other RNA
gccatctttagccgaactaaggaaaagtcctgcaacatttttagcgcccaacgtggaggtcgagaaacggccgtcaaactccaaatggtgatgcaactggaacctctgatgatggccccttctgccgggaacccttaaataggcctctgatggagccctgactgccatttcccccaaacagcaccacctatcagcaggaatcagttaagatcagtcctcgt

SEQ ID NO: 19 - protein, 65 aa, synthetic construct
MNVPKGQTGNSSRGPGDGGNKDHWKESDRKDGKKDQDSRSAPEPKKPEENPASKFSSASNYAALS

SEQ ID NO: 20 - protein, 42 aa, synthetic construct [sequence omitted]

SEQ ID NO: 21 - protein, 53 aa, synthetic construct [sequence omitted]

SEQ ID NO: 22 - protein, 46 aa, synthetic construct
MMTTEEAGTAMKTDMTDGMIGRGAPEMITLGMIIGVMIDVPPKDPN

SEQ ID NO: 23 - protein, 35 aa, synthetic construct
MGIGMAHAGIWMDMVAGIAMMTKAAETMIEAMIPG

SEQ ID NO: 24 - protein, 31 aa, synthetic construct
MAHAGIWMDMVAGIAMMTKAAETMIEAMIPG

SEQ ID NO: 25 - protein, 24 aa, synthetic construct
MDMVAGIAMMTKAAETMIEAMIPG

SEQ ID NO: 26 - protein, 22 aa, synthetic construct
MVAGIAMMTKAAETMIEAMIPG

SEQ ID NO: 27 - protein, 45 aa, synthetic construct
MTTEEAGTAMKTDMTDGMIGRGAPEMITLGMIIGVMIDVPPKDPN

SEQ ID NO: 28 - protein, 36 aa, synthetic construct
MKTDMTDGMIGRGAPEMITLGMIIGVMIDVPPKDPN

SEQ ID NO: 29 - protein, 62 aa, synthetic construct
MYQHVHHYTVIGLGKAEEKQEPASSSYKQKSCLGVVAHACNPSTLGGQSGRITRSGDRDHPG

SEQ ID NO: 30 - protein, 32 aa, synthetic construct
MTDGMIGRGAPEMITLGMIIGVMIDVPPKDPN

SEQ ID NO: 31 - protein, 28 aa, synthetic construct
MIGRGAPEMITLGMIIGVMIDVPPKDPN

SEQ ID NO: 32 - protein, 20 aa, synthetic construct
MITLGMIIGVMIDVPPKDPN

SEQ ID NO: 33 - protein, 67 aa, synthetic construct
MFDTGCSNNKKPPMQMGLKYGWWSGNTSYTRTHGQALTLNVMVVIIRGGAGREQNLSSFAQWQYRSQ

SEQ ID NO: 34 - protein, 51 aa, synthetic construct
MAAEPLVGAECRVCSVNMPGKGIMHVRDRVEKDCARLHHTTQNGTQFRTYK

SEQ ID NO: 35 - protein, 55 aa, synthetic construct
MTWKEMFRQLGTVTMTMCIGCLQLTVPSFPLLHGLLGNPISTGAVFPNRHPTLLF

SEQ ID NO: 36 - protein, 99 aa, synthetic construct [sequence omitted]

SEQ ID NO: 37 - protein, 34 aa, synthetic construct
MPGKGIMHVRDRVEKDCARLHHTTQNGTQFRTYK

SEQ ID NO: 38 - protein, 30 aa, synthetic construct
MLVSKDGAGKPSTTDCKHLNFRRPFSDYYF

SEQ ID NO: 39 - protein, 33 aa, synthetic construct
MPVILALWEAKAGGSRDQEIETILANTVKPRLY

SEQ ID NO: 40 - protein, 54 aa, synthetic construct [sequence omitted]

SEQ ID NO: 41 - protein, 52 aa, synthetic construct
MGLKYGWWSGNTSYTRTHGQALTLNVMVVIIRGGAGREQNLSSFAQWQYRSQ

SEQ ID NO: 42 - protein, 16 aa, synthetic construct
MMTKAAETMIEAMIPG

SEQ ID NO: 43 - protein, 28 aa, synthetic construct
MHVRDRVEKDCARLHHTTQNGTQFRTYK

SEQ ID NO: 44 - protein, 15 aa, synthetic construct
MTKAAETMIEAMIPG

SEQ ID NO: 45 - protein, 28 aa, synthetic construct
MSYNIYMHIERGCEYSCRRASKPKTHRE

SEQ ID NO: 46 - protein, 70 aa, synthetic construct
MKRRNLKTDTPKENAMWRHREKLAIYKPTRIAWNKFFHHTPQKESTLTAPPLQSCSLQNCETIHFCCLRR

SEQ ID NO: 47 - protein, 75 aa, synthetic construct
MVDVLMKRRNLKTDTPKENAMWRHREKLAIYKPTRIAWNKFFHHTPQKESTLTAPPLQSCSLQNCETIHFCCLRR

SEQ ID NO: 48 - protein, 15 aa, synthetic construct
MIIGVMIDVPPKDPN

SEQ ID NO: 49 - protein, 45 aa, synthetic construct
MARLKTVRSSCLDRKATGCSPGSCVRILTALTMPRKGRSCCFIRD

SEQ ID NO: 50 - protein, 46 aa, synthetic construct
MMARLKTVRSSCLDRKATGCSPGSCVRILTALTMPRKGRSCCFIRD

SEQ ID NO: 51 - protein, 30 aa, synthetic construct
MVRSCLYEKYRKYPAEVGGGSLEAWKQRLK

SEQ ID NO: 52 - protein, 31 aa, synthetic construct
MILSLNVEIRGRGKENPMELVAGEALVSLRQ

SEQ ID NO: 53 - protein, 91 aa, synthetic construct
MCSQWPWQNLTKSAPATRPASKDALSRRPLQLSSDCPRDTLSEHCPAKTRQLQNCERRWFHDFLAVVTAVGQLWVTLKGHSDKGHLPACVT

SEQ ID NO: 54 - protein, 93 aa, synthetic construct [sequence omitted]

SEQ ID NO: 55 - protein, 44 aa, synthetic construct
MRPLETHWRAGQTKDNFTDFRRLALISHNLRSQDAGHSKKEKEV

SEQ ID NO: 56 - protein, 64 aa, synthetic construct [sequence omitted]

SEQ ID NO: 57 - protein, 28 aa, synthetic construct
MGTESQFPPLGMKDKVLEVSSDDGYTTM

SEQ ID NO: 58 - protein, 41 aa, synthetic construct [sequence omitted]

SEQ ID NO: 59 - protein, 47 aa, synthetic construct
MTGALCLRSAKPRSEVLTRLHQEQGTRLPRGSWSTEGRDAHKHTMSK

SEQ ID NO: 60 - protein, 69 aa, synthetic construct
MELRIISTTRAGVRQDAQSIHPMTGALCLRSAKPRSEVLTRLHQEQGTRLPRGSWSTEGRDAHKHTMSK

SEQ ID NO: 61 - protein, 68 aa, synthetic construct
MKRAWPPCHSGERQSKTKKTESCSATQAGVEGSGVISAHFNLRLLGSSDSPASASRVAGTTAASLQVS

SEQ ID NO: 62 - protein, 24 aa, synthetic construct
MRSEGQDQPGQYGETLSLLKIQKI

SEQ ID NO: 63 - protein, 19 aa, synthetic construct
MPGLLISTWQHRFMKPLTL

SEQ ID NO: 64 - protein, 16 aa, synthetic construct
MSFLTILANTVKPHLY

SEQ ID NO: 65 - protein, 27 aa, synthetic construct
MSRGRNKLALRSGSIVANEVYPRRDYC

SEQ ID NO: 66 - protein, 12 aa, synthetic construct
MSATLMPSRPEE

SEQ ID NO: 67 - protein, 46 aa, synthetic construct [sequence omitted]

SEQ ID NO: 68 - protein, 34 aa, synthetic construct
MVWTRRCGASPTSYNWGRLTTTVEGTPWNSQTTS

SEQ ID NO: 69 - protein, 20 aa, synthetic construct
MQILEYECWPEIRYFLPSSC

SEQ ID NO: 70 - protein, 27 aa, synthetic construct
MYAKHMGVQVHHPKAMASSVFPKSLRL

SEQ ID NO: 71 - protein, 27 aa, synthetic construct
MQWKLSVLCPAVPSSIQESTPVDERRN

SEQ ID NO: 72 - protein, 21 aa, synthetic construct
MGVLVEEAPMFPNQSAGLMKR

SEQ ID NO: 73 - protein, 31 aa, synthetic construct
MGLGHVPTCSSLYSDWTWKGRREARASILIL

SEQ ID NO: 74 - protein, 33 aa, synthetic construct
MKSVEVRPLDALAWKSHILLAKANHKATTNSRR

SEQ ID NO: 75 - protein, 40 aa, synthetic construct
MTARFKRMKSVEVRPLDALAWKSHILLAKANHKATTNSRR

SEQ ID NO: 76 - protein, 47 aa, synthetic construct
MIKVKESKFTTLLVFSFYPGCELNKKSAAVAHACNPSPWGGRGGRIT

SEQ ID NO: 77 - protein, 27 aa, synthetic construct
MLARLVSNSRPQVIRQPRPPKMLGLQA

SEQ ID NO: 78 - protein, 17 aa, synthetic construct
MKDKVLEVSSDDGYTTM

SEQ ID NO: 79 - protein, 21 aa, synthetic construct
MKARAVAKGTSPSGEASSAQL

SEQ ID NO: 80 - protein, 10 aa, synthetic construct
MDGFLEEEAR

SEQ ID NO: 81 - protein, 23 aa, synthetic construct
MREHRGEAPTLGFMDGFLEEEAR

SEQ ID NO: 82 - protein, 66 aa, synthetic construct
MSLLIRECLSSLYLNFSKRENAFRTSNSDGSRVFLAALFLNEDSPGGSLCCRDTQISPCSCSFQSF

SEQ ID NO: 83 - protein, 18 aa, synthetic construct
MMKPRYTAYLAFRQGKPA

SEQ ID NO: 84 - protein, 55 aa, synthetic construct
MWRHREKLAIYKPTRIAWNKFFHHTPQKESTLTAPPLQSCSLQNCETIHFCCLRR

SEQ ID NO: 85 - protein, 28 aa, synthetic construct
MPDQDWAQPPALQVDRLRSAASEAAWDG

SEQ ID NO: 86 - protein, 9 aa, synthetic construct
MMRKEMRPA

SEQ ID NO: 87 - protein, 14 aa, synthetic construct
MELVAGEALVSLRQ

SEQ ID NO: 88 - protein, 18 aa, synthetic construct
MEKRSQAKTAVGQSFGET

SEQ ID NO: 89 - protein, 32 aa, synthetic construct
MGNNTLEWSGNCWPLSPAVLPEGNPNRRSDSQ

SEQ ID NO: 90 - protein, 29 aa, synthetic construct [sequence omitted]

SEQ ID NO: 91 - protein, 27 aa, synthetic construct
MQKMEATGRGWESLGFRKEAPGSPVLL

SEQ ID NO: 92 - protein, 8 aa, synthetic construct
MSFWRETE

SEQ ID NO: 93 - protein, 11 aa, synthetic construct
MRKLFGNCVTV

SEQ ID NO: 94 - protein, 8 aa, synthetic construct
MAPSAGNP

SEQ ID NO: 95 - protein, 32 aa, synthetic construct
MSDRREEEGNVEWVASILIKKGTDLPSTVRIT

SEQ ID NO: 96 - protein, 27 aa, synthetic construct
MGAVCEALRQYSPGGFQGSRAASVFSR

SEQ ID NO: 97 - protein, 54 aa, synthetic construct
MDSAPEEENLETLRLSETYSQLPKLKMFVAGSGTSGFRAGTFIAPVMKKRMKCG

SEQ ID NO: 98 - protein, 11 aa, synthetic construct
MYQHVHHYTVI

SEQ ID NO: 99 - protein, 9 aa, synthetic construct
KLFGNCVTV

SEQ ID NO: 100 - protein, 11 aa, synthetic construct
LNFRRPFSDYY

SEQ ID NO: 101 - protein, 11 aa, synthetic construct
SFLTILANTVK

SEQ ID NO: 102 - protein, 11 aa, synthetic construct
LISEDPFLITI

SEQ ID NO: 103 - protein, 11 aa, synthetic construct
YTAYLAFRQGK

SEQ ID NO: 104 - protein, 11 aa, synthetic construct
LISTWQHRFMK

SEQ ID NO: 105 - protein, 11 aa, synthetic construct
QILEYECWPEI

SEQ ID NO: 106 - protein, 11 aa, synthetic construct
MAHAGIWMDMV

SEQ ID NO: 107 - protein, 11 aa, synthetic construct
MAHAGIWMDMV

SEQ ID NO: 108 - protein, 11 aa, synthetic construct
MAHAGIWMDMV

SEQ ID NO: 109 - protein, 11 aa, synthetic construct
MAHAGIWMDMV

SEQ ID NO: 110 - protein, 9 aa, synthetic construct
ILISEDPFL

SEQ ID NO: 111 - protein, 11 aa, synthetic construct
STWQHRFMKPL

SEQ ID NO: 112 - protein, 11 aa, synthetic construct
STYVSKPVSWA

SEQ ID NO: 113 - protein, 11 aa, synthetic construct
KTVRSSCLDRK

SEQ ID NO: 114 - protein, 11 aa, synthetic construct
KTVRSSCLDRK

SEQ ID NO: 115 - protein, 11 aa, synthetic construct
IIGVMIDVPPK

SEQ ID NO: 116 - protein, 11 aa, synthetic construct
IIGVMIDVPPK

SEQ ID NO: 117 - protein, 11 aa, synthetic construct
IIGVMIDVPPK

SEQ ID NO: 118 - protein, 11 aa, synthetic construct
IIGVMIDVPPK

SEQ ID NO: 119 - protein, 11 aa, synthetic construct
IIGVMIDVPPK

SEQ ID NO: 120 - protein, 11 aa, synthetic construct
IIGVMIDVPPK

SEQ ID NO: 121 - protein, 11 aa, synthetic construct
IIGVMIDVPPK

SEQ ID NO: 122 - protein, 11 aa, synthetic construct
SIHPMTGALCL

SEQ ID NO: 123 - protein, 9 aa, synthetic construct
MIIGVMIDV

SEQ ID NO: 124 - protein, 9 aa, synthetic construct
MIIGVMIDV

SEQ ID NO: 125 - protein, 9 aa, synthetic construct
MIIGVMIDV

SEQ ID NO: 126 - protein, 9 aa, synthetic construct
MIIGVMIDV

SEQ ID NO: 127 - protein, 9 aa, synthetic construct
MIIGVMIDV

SEQ ID NO: 128 - protein, 9 aa, synthetic construct
MIIGVMIDV

SEQ ID NO: 129 - protein, 9 aa, synthetic construct
MIIGVMIDV

SEQ ID NO: 130 - protein, 11 aa, synthetic construct
APTLGFMDGFL

SEQ ID NO: 131 - protein, 11 aa, synthetic construct
GQALTLNVMVV

SEQ ID NO: 132 - protein, 11 aa, synthetic construct
GQALTLNVMVV

SEQ ID NO: 133 - protein, 11 aa, synthetic construct
GQALTLNVMVV

SEQ ID NO: 134 - protein, 11 aa, synthetic construct
SYNWGRLTTTV

SEQ ID NO: 135 - protein, 11 aa, synthetic construct
ITISKDVHIVL

SEQ ID NO: 136 - protein, 11 aa, synthetic construct
MVQENQVQLIV

SEQ ID NO: 137 - protein, 11 aa, synthetic construct
GFHQVLFFQKK

SEQ ID NO: 138 - protein, 9 aa, synthetic construct
FLTILANTV

SEQ ID NO: 139 - protein, 11 aa, synthetic construct
RRWFHDFLAVV

SEQ ID NO: 140 - protein, 11 aa, synthetic construct
RRWFHDFLAVV

SEQ ID NO: 141 - protein, 11 aa, synthetic construct
TSYTRTHGQAL

SEQ ID NO: 142 - protein, 11 aa, synthetic construct
TSYTRTHGQAL

SEQ ID NO: 143 - protein, 11 aa, synthetic construct
TSYTRTHGQAL

SEQ ID NO: 144 - protein, 11 aa, synthetic construct
WMDMVAGIAMM

SEQ ID NO: 145 - protein, 11 aa, synthetic construct
WMDMVAGIAMM

SEQ ID NO: 146 - protein, 11 aa, synthetic construct
WMDMVAGIAMM

SEQ ID NO: 147 - protein, 11 aa, synthetic construct
WMDMVAGIAMM

SEQ ID NO: 148 - protein, 11 aa, synthetic construct
IYKPTRIAWNK

SEQ ID NO: 149 - protein, 11 aa, synthetic construct
IYKPTRIAWNK

SEQ ID NO: 150 - protein, 11 aa, synthetic construct
IYKPTRIAWNK

SEQ ID NO: 151 - protein, 11 aa, synthetic construct
KFTTLLVFSFY

SEQ ID NO: 152 - protein, 11 aa, synthetic construct
CLYEKYRKYPA

SEQ ID NO: 153 - protein, 9 aa, synthetic construct
ALTLNVMVV

SEQ ID NO: 154 - protein, 9 aa, synthetic construct
ALTLNVMVV

SEQ ID NO: 155 - protein, 9 aa, synthetic construct
ALTLNVMVV

SEQ ID NO: 156 - protein, 11 aa, synthetic construct
FSFYPGCELNK

SEQ ID NO: 157 - protein, 11 aa, synthetic construct
AVVTAVGQLWV

SEQ ID NO: 158 - protein, 11 aa, synthetic construct
AVVTAVGQLWV

SEQ ID NO: 159 - protein, 11 aa, synthetic construct
AMMTKAAETMI

SEQ ID NO: 160 - protein, 11 aa, synthetic construct
AMMTKAAETMI

SEQ ID NO: 161 - protein, 11 aa, synthetic construct
AMMTKAAETMI

SEQ ID NO: 162 - protein, 11 aa, synthetic construct
AMMTKAAETMI

SEQ ID NO: 163 - protein, 11 aa, synthetic construct
AMMTKAAETMI

SEQ ID NO: 164 - protein, 11 aa, synthetic construct
AMMTKAAETMI

SEQ ID NO: 165 - protein, 11 aa, synthetic construct
DPFLITISKDV

SEQ ID NO: 166 - protein, 11 aa, synthetic construct
ETLSLLKIQKI

SEQ ID NO: 167 - protein, 10 aa, synthetic construct
NFTDFRRLAL

SEQ ID NO: 168 - protein, 11 aa, synthetic construct
FTDFRRLALIS

SEQ ID NO: 169 - protein, 11 aa, synthetic construct
KLAIYKPTRIA

SEQ ID NO: 170 - protein, 11 aa, synthetic construct
KLAIYKPTRIA

SEQ ID NO: 171 - protein, 11 aa, synthetic construct
KLAIYKPTRIA

SEQ ID NO: 172 - protein, 9 aa, synthetic construct
VMIQTGIGM

SEQ ID NO: 173 - protein, 9 aa, synthetic construct
LISEDPFLI

SEQ ID NO: 174 - protein, 11 aa, synthetic construct
NFTDFRRLALI

SEQ ID NO: 175 - protein, 11 aa, synthetic construct
ALETSIGIVMI

SEQ ID NO: 176 - protein, 10 aa, synthetic construct
SYTRTHGQAL

SEQ ID NO: 177 - protein, 10 aa, synthetic construct
SYTRTHGQAL

SEQ ID NO: 178 - protein, 10 aa, synthetic construct
SYTRTHGQAL

SEQ ID NO: 179 - protein, 11 aa, synthetic construct
LTLNVMVVIIR

SEQ ID NO: 180 - protein, 11 aa, synthetic construct
LTLNVMVVIIR

SEQ ID NO: 181 - protein, 11 aa, synthetic construct
LTLNVMVVIIR

SEQ ID NO: 182 - protein, 11 aa, synthetic construct
KFSSASNYAAL

SEQ ID NO: 183 - protein, 11 aa, synthetic construct
VNMPGKGIMHV

SEQ ID NO: 184 - protein, 11 aa, synthetic construct
RILTALTMPRK

SEQ ID NO: 185 - protein, 11 aa, synthetic construct
RILTALTMPRK

SEQ ID NO: 186 - protein, 11 aa, synthetic construct
TFIAPVMKKRM

SEQ ID NO: 187 - protein, 11 aa, synthetic construct
ANEVYPRRDYC

SEQ ID NO: 188 - protein, 11 aa, synthetic construct
VMIQTGIGMGI

SEQ ID NO: 189 - protein, 11 aa, synthetic construct
EMFRQLGTVTM

SEQ ID NO: 190 - protein, 11 aa, synthetic construct
EMFRQLGTVTM

SEQ ID NO: 191 - protein, 11 aa, synthetic construct
GIMHVRDRVEK

SEQ ID NO: 192 - protein, 11 aa, synthetic construct
GIMHVRDRVEK

SEQ ID NO: 193 - protein, 11 aa, synthetic construct
VHHYTVIGLGK

SEQ ID NO: 194 - protein, 11 aa, synthetic construct
TTVEGTPWNSQ

SEQ ID NO: 195 - protein, 11 aa, synthetic construct
APATRPASKDA

SEQ ID NO: 196 - protein, 11 aa, synthetic construct
APATRPASKDA

SEQ ID NO: 197 - protein, 11 aa, synthetic construct
KYGWWSGNTSY

SEQ ID NO: 198 - protein, 11 aa, synthetic construct
KYGWWSGNTSY

SEQ ID NO: 199 - protein, 11 aa, synthetic construct
KYGWWSGNTSY

SEQ ID NO: 200 - protein, 11 aa, synthetic construct
TYSQLPKLKMF

SEQ ID NO: 201 - protein, 11 aa, synthetic construct
GLLGNPISTGA

SEQ ID NO: 202 - protein, 11 aa, synthetic construct
GLLGNPISTGA

SEQ ID NO: 203 - protein, 11 aa, synthetic construct
QLWELNQETQI

SEQ ID NO: 204 - protein, 11 aa, synthetic construct
GFRAGTFIAPV

SEQ ID NO: 205 - protein, 11 aa, synthetic construct
TQNGTQFRTYK

SEQ ID NO: 206 - protein, 11 aa, synthetic construct
TQNGTQFRTYK

SEQ ID NO: 207 - protein, 11 aa, synthetic construct
TQNGTQFRTYK

SEQ ID NO: 208 - protein, 11 aa, synthetic construct
LTILANTVKPH

SEQ ID NO: 209 - protein, 11 aa, synthetic construct
AVFPNRHPTLL

SEQ ID NO: 210 - protein, 11 aa, synthetic construct
AVFPNRHPTLL

SEQ ID NO: 211 - protein, 8 aa, synthetic construct
SASNYAAL

SEQ ID NO: 212 - protein, 11 aa, synthetic construct
KPTRIAWNKFF

SEQ ID NO: 213 - protein, 11 aa, synthetic construct
KPTRIAWNKFF

SEQ ID NO: 214 - protein, 11 aa, synthetic construct
KPTRIAWNKFF

SEQ ID NO: 215 - protein, 11 aa, synthetic construct
ASSVFPKSLRL

SEQ ID NO: 216 - protein, 11 aa, synthetic construct
MTTEEAGTAMK

SEQ ID NO: 217 - protein, 11 aa, synthetic construct
MTTEEAGTAMK

SEQ ID NO: 218 - protein, 8 aa, synthetic construct
FHDFLAVV

SEQ ID NO: 219 - protein, 8 aa, synthetic construct
FHDFLAVV

SEQ ID NO: 220 - protein, 11 aa, synthetic construct
MIALETSIGIV

SEQ ID NO: 221 - protein, 11 aa, synthetic construct
NFRRPFSDYYF

SEQ ID NO: 222 - protein, 11 aa, synthetic construct
EMITLGMIIGV

SEQ ID NO: 223 - protein, 11 aa, synthetic construct
EMITLGMIIGV

SEQ ID NO: 224 - protein, 11 aa, synthetic construct
EMITLGMIIGV

SEQ ID NO: 225 - protein, 11 aa, synthetic construct
EMITLGMIIGV

SEQ ID NO: 226 - protein, 11 aa, synthetic construct
EMITLGMIIGV

SEQ ID NO: 227 - protein, 11 aa, synthetic construct
FRQLGTVTMTM

SEQ ID NO: 228 - protein, 11 aa, synthetic construct
FRQLGTVTMTM

SEQ ID NO: 229 - protein, 11 aa, synthetic construct
GAPEMITLGMI

SEQ ID NO: 230 - protein, 11 aa, synthetic construct
GAPEMITLGMI

SEQ ID NO: 231 - protein, 11 aa, synthetic construct
GAPEMITLGMI

SEQ ID NO: 232 - protein, 11 aa, synthetic construct
GAPEMITLGMI

SEQ ID NO: 233 - protein, 11 aa, synthetic construct
GAPEMITLGMI

SEQ ID NO: 234 - protein, 11 aa, synthetic construct
FSFVLVRRPSR

SEQ ID NO: 235 - protein, 11 aa, synthetic construct
EIETILANTVK

SEQ ID NO: 236 - protein, 11 aa, synthetic construct
FIAPVMKKRMK

SEQ ID NO: 237 - protein, 11 aa, synthetic construct
SQFPPLGMKDK

SEQ ID NO: 238 - protein, 11 aa, synthetic construct
FGFHQVLFFQK

SEQ ID NO: 239 - protein, 11 aa, synthetic construct
MSYNIYMHIER

SEQ ID NO: 240 - protein, 11 aa, synthetic construct
ISKDVHIVLRL

SEQ ID NO: 241 - protein, 11 aa, synthetic construct
EYECWPEIRYF

SEQ ID NO: 242 - protein, 11 aa, synthetic construct
ISTTRAGVRQD

SEQ ID NO: 243 - protein, 11 aa, synthetic construct
GTDLPSTVRIT

SEQ ID NO: 244 - protein, 11 aa, synthetic construct
TAVGQLWVTLK

SEQ ID NO: 245 - protein, 11 aa, synthetic construct
TAVGQLWVTLK

SEQ ID NO: 246 - protein, 11 aa, synthetic construct
GMAHAGIWMDM

SEQ ID NO: 247 - protein, 11 aa, synthetic construct
GMAHAGIWMDM

SEQ ID NO: 248 - protein, 11 aa, synthetic construct
GMAHAGIWMDM

SEQ ID NO: 249 - protein, 11 aa, synthetic construct
GTFIAPVMKKR

SEQ ID NO: 250 - protein, 11 aa, synthetic construct
IWMDMVAGIAM

SEQ ID NO: 251 - protein, 11 aa, synthetic construct
IWMDMVAGIAM

SEQ ID NO: 252 - protein, 11 aa, synthetic construct
IWMDMVAGIAM

SEQ ID NO: 253 - protein, 11 aa, synthetic construct
IWMDMVAGIAM

SEQ ID NO: 254 - protein, 11 aa, synthetic construct
YEKYRKYPAEV

SEQ ID NO: 255 - protein, 8 aa, synthetic construct
LISEDPFL

SEQ ID NO: 256 - protein, 11 aa, synthetic construct
KLALRSGSIVA

SEQ ID NO: 257 - protein, 11 aa, synthetic construct
APEMITLGMII

SEQ ID NO: 258 - protein, 11 aa, synthetic construct
APEMITLGMII

SEQ ID NO: 259 - protein, 11 aa, synthetic construct
APEMITLGMII

SEQ ID NO: 260 - protein, 11 aa, synthetic construct
APEMITLGMII

SEQ ID NO: 261 - protein, 11 aa, synthetic construct
APEMITLGMII

SEQ ID NO: 262 - protein, 8 aa, synthetic construct
FLAVVTAV

SEQ ID NO: 263 - protein, 8 aa, synthetic construct
FLAVVTAV

SEQ ID NO: 264 - protein, 11 aa, synthetic construct
AMKTDMTDGMI

SEQ ID NO: 265 - protein, 11 aa, synthetic construct
AMKTDMTDGMI

SEQ ID NO: 266 - protein, 11 aa, synthetic construct
PMFPNQSAGLM

SEQ ID NO: 267 - protein, 11 aa, synthetic construct
GVISAHFNLRL

SEQ ID NO: 268 - protein, 11 aa, synthetic construct
KHMGVQVHHPK

SEQ ID NO: 269 - protein, 11 aa, synthetic construct
DMVAGIAMMTK

SEQ ID NO: 270 - protein, 11 aa, synthetic construct
DMVAGIAMMTK

SEQ ID NO: 271 - protein, 11 aa, synthetic construct
DMVAGIAMMTK

SEQ ID NO: 272 - protein, 11 aa, synthetic construct
DMVAGIAMMTK

SEQ ID NO: 273 - protein, 11 aa, synthetic construct
DMVAGIAMMTK

SEQ ID NO: 274 - protein, 9 aa, synthetic construct
SSASNYAAL

SEQ ID NO: 275 - protein, 11 aa, synthetic construct
TTQNGTQFRTY

SEQ ID NO: 276 - protein, 11 aa, synthetic construct
TTQNGTQFRTY

SEQ ID NO: 277 - protein, 11 aa, synthetic construct
TTQNGTQFRTY

SEQ ID NO: 278 - protein, 11 aa, synthetic construct
GQTKDNFTDFR

SEQ ID NO: 279 - protein, 11 aa, synthetic construct
ASPTSYNWGRL

SEQ ID NO: 280 - protein, 11 aa, synthetic construct
AQSIHPMTGAL

SEQ ID NO: 281 - protein, 9 aa, synthetic construct
DFLAVVTAV

SEQ ID NO: 282 - protein, 9 aa, synthetic construct
DFLAVVTAV

SEQ ID NO: 283 - protein, 11 aa, synthetic construct
VPSFPLLHGLL

SEQ ID NO: 284 - protein, 11 aa, synthetic construct
VPSFPLLHGLL

SEQ ID NO: 285 - protein, 11 aa, synthetic construct
VDVLMKRRNLK

SEQ ID NO: 286 - protein, 8 aa, synthetic construct
VISAHFNL

SEQ ID NO: 287 - protein, 11 aa, synthetic construct
PQVIRQPRPPK

SEQ ID NO: 288 - protein, 11 aa, synthetic construct
PPMQMGLKYGW

SEQ ID NO: 289 - protein, 11 aa, synthetic construct
LLIRECLSSLY

SEQ ID NO: 290 - protein, 8 aa, synthetic construct
ISEDPFLI

SEQ ID NO: 291 - protein, 11 aa, synthetic construct
LWVTLKGHSDK

SEQ ID NO: 292 - protein, 11 aa, synthetic construct
LWVTLKGHSDK

SEQ ID NO: 293 - protein, 11 aa, synthetic construct
GTESQFPPLGM

SEQ ID NO: 294 - protein, 11 aa, synthetic construct
MPVILALWEAK

SEQ ID NO: 295 - protein, 11 aa, synthetic construct
SHPEGHLTRPL

SEQ ID NO: 296 - protein, 11 aa, synthetic construct
LRSGSIVANEV

SEQ ID NO: 297 - protein, 11 aa, synthetic construct
VPSSIQESTPV

SEQ ID NO: 298 - protein, 11 aa, synthetic construct
MFVAGSGTSGF

SEQ ID NO: 299 - protein, 10 aa, synthetic construct
YMHIERGCEY

SEQ ID NO: 300 - protein, 11 aa, synthetic construct
QYGETLSLLKI

SEQ ID NO: 301 - protein, 11 aa, synthetic construct
AMASSVFPKSL

SEQ ID NO: 302 - protein, 11 aa, synthetic construct
PISTGAVFPNR

SEQ ID NO: 303 - protein, 11 aa, synthetic construct
PISTGAVFPNR

SEQ ID NO: 304 - protein, 11 aa, synthetic construct
STLGGQSGRIT

SEQ ID NO: 305 - protein, 11 aa, synthetic construct
KVLEVSSDDGY

SEQ ID NO: 306 - protein, 11 aa, synthetic construct
KVLEVSSDDGY

SEQ ID NO: 307 - protein, 11 aa, synthetic construct
KAAETMIEAMI

SEQ ID NO: 308 - protein, 11 aa, synthetic construct
KAAETMIEAMI

SEQ ID NO: 309 - protein, 11 aa, synthetic construct
KAAETMIEAMI

SEQ ID NO: 310 - protein, 11 aa, synthetic construct
KAAETMIEAMI

SEQ ID NO: 311 - protein, 11 aa, synthetic construct
KAAETMIEAMI

SEQ ID NO: 312 - protein, 11 aa, synthetic construct
KAAETMIEAMI

SEQ ID NO: 313 - protein, 11 aa, synthetic construct
KAAETMIEAMI

SEQ ID NO: 314 - protein, 11 aa, synthetic construct
KAAETMIEAMI

SEQ ID NO: 315 - protein, 11 aa, synthetic construct
RWFHDFLAVVT

SEQ ID NO: 316 - protein, 11 aa, synthetic construct
RWFHDFLAVVT

SEQ ID NO: 317 - protein, 11 aa, synthetic construct
QSGRITRSGDR

SEQ ID NO: 318 - protein, 10 aa, synthetic construct
MFPNQSAGLM

SEQ ID NO: 319 - protein, 11 aa, synthetic construct
AMWRHREKLAI

SEQ ID NO: 320 - protein, 11 aa, synthetic construct
AMWRHREKLAI

SEQ ID NO: 321 - protein, 11 aa, synthetic construct
ALAWKSHILLA

SEQ ID NO: 322 - protein, 11 aa, synthetic construct
ALAWKSHILLA

SEQ ID NO: 323 - protein, 11 aa, synthetic construct
FLITISKDVHI

SEQ ID NO: 324 - protein, 11 aa, synthetic construct
SHILLAKANHK

SEQ ID NO: 325 - protein, 11 aa, synthetic construct
SHILLAKANHK

SEQ ID NO: 326 - protein, 11 aa, synthetic construct
FRAGTFIAPVM

SEQ ID NO: 327 - protein, 11 aa, synthetic construct
LYSDWTWKGRR

SEQ ID NO: 328 - protein, 11 aa, synthetic construct
SIVANEVYPRR

SEQ ID NO: 329 - protein, 11 aa, synthetic construct
EEGNVEWVASI

SEQ ID NO: 330 - protein, 11 aa, synthetic construct
GTGGGSTYVSK

SEQ ID NO: 331 - protein, 11 aa, synthetic construct
NVEWVASILIK

SEQ ID NO: 332 - protein, 11 aa, synthetic construct
GSIVANEVYPR

SEQ ID NO: 333 - protein, 11 aa, synthetic construct
VSWADETMTWK

SEQ ID NO: 334 - protein, 11 aa, synthetic construct
QNLSSFAQWQY

SEQ ID NO: 335 - protein, 11 aa, synthetic construct
QNLSSFAQWQY

SEQ ID NO: 336 - protein, 11 aa, synthetic construct
QNLSSFAQWQY

SEQ ID NO: 337 - protein, 8 aa, synthetic construct
EEGNVEWV

SEQ ID NO: 338 - protein, 11 aa, synthetic construct
RTSNSDGSRVF

SEQ ID NO: 339 - protein, 11 aa, synthetic construct
GHLTRPLEQTK

SEQ ID NO: 340 - protein, 10 aa, synthetic construct
SWADETMTWK

SEQ ID NO: 341 - protein, 11 aa, synthetic construct
IALETSIGIVM

SEQ ID NO: 342 - protein, 11 aa, synthetic construct
STTDCKHLNFR

SEQ ID NO: 343 - protein, 11 aa, synthetic construct
RLVSNSRPQVI

SEQ ID NO: 344 - protein, 11 aa, synthetic construct
KPVSWADETMT

SEQ ID NO: 345 - protein, 9 aa, synthetic construct
GVISAHFNL

SEQ ID NO: 346 - protein, 11 aa, synthetic construct
RTHGQALTLNV

SEQ ID NO: 347 - protein, 11 aa, synthetic construct
RTHGQALTLNV

SEQ ID NO: 348 - protein, 11 aa, synthetic construct
RTHGQALTLNV

SEQ ID NO: 349 - protein, 11 aa, synthetic construct
TAMKTDMTDGM

SEQ ID NO: 350 - protein, 11 aa, synthetic construct
TAMKTDMTDGM

SEQ ID NO: 351 - protein, 10 aa, synthetic construct
SEDPFLITIS

SEQ ID NO: 352 - protein, 8 aa, synthetic construct
LLGNPIST

SEQ ID NO: 353 - protein, 8 aa, synthetic construct
LLGNPIST

SEQ ID NO: 354 - protein, 11 aa, synthetic construct
QENQVQLIVSI

SEQ ID NO: 355 - protein, 11 aa, synthetic construct
NSDGSRVFLAA

SEQ ID NO: 356 - protein, 11 aa, synthetic construct
TSNSDGSRVFL

SEQ ID NO: 357 - protein, 8 aa, synthetic construct
AIYKPTRI

SEQ ID NO: 358 - protein, 8 aa, synthetic construct
AIYKPTRI

SEQ ID NO: 359 - protein, 8 aa, synthetic construct
AIYKPTRI

SEQ ID NO: 360 - protein, 11 aa, synthetic construct
SFYPGCELNKK

SEQ ID NO: 361 - protein, 11 aa, synthetic construct
FLAVVTAVGQL

SEQ ID NO: 362 - protein, 11 aa, synthetic construct
FLAVVTAVGQL

SEQ ID NO: 363 - protein, 9 aa, synthetic construct
EMITLGMII

SEQ ID NO: 364 - protein, 9 aa, synthetic construct
EMITLGMII

SEQ ID NO: 365 - protein, 9 aa, synthetic construct
EMITLGMII

SEQ ID NO: 366 - protein, 9 aa, synthetic construct
EMITLGMII

SEQ ID NO: 367 - protein, 9 aa, synthetic construct
EMITLGMII

SEQ ID NO: 368 - protein, 9 aa, synthetic construct
VLVEEAPMF

SEQ ID NO: 369 - protein, 11 aa, synthetic construct
LTALTMPRKGR

SEQ ID NO: 370 - protein, 11 aa, synthetic construct
LTALTMPRKGR

SEQ ID NO: 371 - protein, 11 aa, synthetic construct
LTAPPLQSCSL

SEQ ID NO: 372 - protein, 11 aa, synthetic construct
LTAPPLQSCSL

SEQ ID NO: 373 - protein, 11 aa, synthetic construct
LTAPPLQSCSL

SEQ ID NO: 374 - protein, 11 aa, synthetic construct
GSLEAWKQRLK

SEQ ID NO: 375 - protein, 11 aa, synthetic construct
REFGFHQVLFF

SEQ ID NO: 376 - protein, 8 aa, synthetic construct
ALAWKSHI

SEQ ID NO: 377 - protein, 8 aa, synthetic construct
ALAWKSHI

SEQ ID NO: 378 - protein, 11 aa, synthetic construct
MMTTEEAGTAM

SEQ ID NO: 379 - protein, 11 aa, synthetic construct
GMIGRGAPEMI

SEQ ID NO: 380 - protein, 11 aa, synthetic construct
GMIGRGAPEMI

SEQ ID NO: 381 - protein, 11 aa, synthetic construct
GMIGRGAPEMI

SEQ ID NO: 382 - protein, 11 aa, synthetic construct
GMIGRGAPEMI

SEQ ID NO: 383 - protein, 9 aa, synthetic construct
IWMDMVAGI

SEQ ID NO: 384 - protein, 9 aa, synthetic construct
IWMDMVAGI

SEQ ID NO: 385 - protein, 9 aa, synthetic construct
IWMDMVAGI

SEQ ID NO: 386 - protein, 9 aa, synthetic construct
IWMDMVAGI

SEQ ID NO: 387 - protein, 9 aa, synthetic construct
FLITISKDV

SEQ ID NO: 388 - protein, 11 aa, synthetic construct
QTKDNFTDFRR

SEQ ID NO: 389 - protein, 11 aa, synthetic construct
SLNVEIRGRGK

SEQ ID NO: 390 - protein, 11 aa, synthetic construct
DALAWKSHILL

SEQ ID NO: 391 - protein, 11 aa, synthetic construct
DALAWKSHILL

SEQ ID NO: 392 - protein, 11 aa, synthetic construct
SSDSPASASRV

SEQ ID NO: 393 - protein, 11 aa, synthetic construct
MVAGIAMMTKA

SEQ ID NO: 394 - protein, 11 aa, synthetic construct
MVAGIAMMTKA

SEQ ID NO: 395 - protein, 11 aa, synthetic construct
MVAGIAMMTKA

SEQ ID NO: 396 - protein, 11 aa, synthetic construct
MVAGIAMMTKA

SEQ ID NO: 397 - protein, 11 aa, synthetic construct
MVAGIAMMTKA

SEQ ID NO: 398 - protein, 11 aa, synthetic construct
MVAGIAMMTKA

SEQ ID NO: 399 - protein, 11 aa, synthetic construct
MPDQDWAQPPA

SEQ ID NO: 400 - protein, 11 aa, synthetic construct
GGFQGSRAASV

SEQ ID NO: 401 - protein, 11 aa, synthetic construct
LAIYKPTRIAW

SEQ ID NO: 402 - protein, 11 aa, synthetic construct
LAIYKPTRIAW

SEQ ID NO: 403 - protein, 11 aa, synthetic construct
LAIYKPTRIAW

SEQ ID NO: 404 - protein, 11 aa, synthetic construct
MTDGMIGRGAP

SEQ ID NO: 405 - protein, 11 aa, synthetic construct
MTDGMIGRGAP

SEQ ID NO: 406 - protein, 11 aa, synthetic construct
MTDGMIGRGAP

SEQ ID NO: 407 - protein, 11 aa, synthetic construct
MTDGMIGRGAP

SEQ ID NO: 408 - protein, 8 aa, synthetic construct
HVHHYTVI

SEQ ID NO: 409 - protein, 9 aa, synthetic construct
GLLGNPIST

SEQ ID NO: 410 - protein, 9 aa, synthetic construct
GLLGNPIST

SEQ ID NO: 411 - protein, 8 aa, synthetic construct
MYAKHMGV

SEQ ID NO: 412 - protein, 11 aa, synthetic construct
RAGTFIAPVMK

SEQ ID NO: 413 - protein, 8 aa, synthetic construct
TKDNFTDF

SEQ ID NO: 414 - protein, 11 aa, synthetic construct
LSSLYLNFSKR

SEQ ID NO: 415 - protein, 11 aa, synthetic construct
PSREFGFHQVL

SEQ ID NO: 416 - protein, 11 aa, synthetic construct
GASPTSYNWGR

SEQ ID NO: 417 - protein, 11 aa, synthetic construct
DVHIVLRLLLL

SEQ ID NO: 418 - protein, 11 aa, synthetic construct
ENGFSFVLVRR

SEQ ID NO: 419 - protein, 11 aa, synthetic construct
AQEENGFSFVL

SEQ ID NO: 420 - protein, 11 aa, synthetic construct
KTDMTDGMIGR

SEQ ID NO: 421 - protein, 11 aa, synthetic construct
KTDMTDGMIGR

SEQ ID NO: 422 - protein, 11 aa, synthetic construct
KTDMTDGMIGR

SEQ ID NO: 423 - protein, 11 aa, synthetic construct
EVSSDDGYTTM

SEQ ID NO: 424 - protein, 11 aa, synthetic construct
EVSSDDGYTTM

SEQ ID NO: 425 - protein, 8 aa, synthetic construct
MVAGIAMM

SEQ ID NO: 426 - protein, 8 aa, synthetic construct
MVAGIAMM

SEQ ID NO: 427 - protein, 8 aa, synthetic construct
MVAGIAMM

SEQ ID NO: 428 - protein, 8 aa, synthetic construct
MVAGIAMM

SEQ ID NO: 429 - protein, 8 aa, synthetic construct
MVAGIAMM

SEQ ID NO: 430 - protein, 8 aa, synthetic construct
MVAGIAMM

SEQ ID NO: 431 - protein, 11 aa, synthetic construct
ALQVDRLRSAA

SEQ ID NO: 432 - protein, 11 aa, synthetic construct
LGNPISTGAVF

SEQ ID NO: 433 - protein, 11 aa, synthetic construct
LGNPISTGAVF

SEQ ID NO: 434 - protein, 11 aa, synthetic construct
AGTFIAPVMKK

SEQ ID NO: 435 - protein, 9 aa, synthetic construct
GMKDKVLEV

SEQ ID NO: 436 - protein, 10 aa, synthetic construct
GFQGSRAASV

SEQ ID NO: 437 - protein, 11 aa, synthetic construct
SSRGPGDGGNK

SEQ ID NO: 438 - protein, 11 aa, synthetic construct
RGAPEMITLGM

SEQ ID NO: 439 - protein, 11 aa, synthetic construct
RGAPEMITLGM

SEQ ID NO: 440 - protein, 11 aa, synthetic construct
RGAPEMITLGM

SEQ ID NO: 441 - protein, 11 aa, synthetic construct
RGAPEMITLGM

SEQ ID NO: 442 - protein, 11 aa, synthetic construct
RGAPEMITLGM

SEQ ID NO: 443 - protein, 11 aa, synthetic construct
GWWSGNTSYTR

SEQ ID NO: 444 - protein, 11 aa, synthetic construct
GWWSGNTSYTR

SEQ ID NO: 445 - protein, 11 aa, synthetic construct
GWWSGNTSYTR

SEQ ID NO: 446 - protein, 11 aa, synthetic construct
EAQEENGFSFV

SEQ ID NO: 447 - protein, 9 aa, synthetic construct
VEWVASILI

SEQ ID NO: 448 - protein, 11 aa, synthetic construct
DGMIGRGAPEM

SEQ ID NO: 449 - protein, 11 aa, synthetic construct
DGMIGRGAPEM

SEQ ID NO: 450 - protein, 11 aa, synthetic construct
DGMIGRGAPEM

SEQ ID NO: 451 - protein, 11 aa, synthetic construct
DGMIGRGAPEM

SEQ ID NO: 452 - protein, 11 aa, synthetic construct
VHIVLRLLLLK

SEQ ID NO: 453 - protein, 9 aa, synthetic construct
DMVAGIAMM

SEQ ID NO: 454 - protein, 9 aa, synthetic construct
DMVAGIAMM

SEQ ID NO: 455 - protein, 9 aa, synthetic construct
DMVAGIAMM

SEQ ID NO: 456 - protein, 9 aa, synthetic construct
DMVAGIAMM

SEQ ID NO: 457 - protein, 9 aa, synthetic construct
DMVAGIAMM

SEQ ID NO: 458 - protein, 11 aa, synthetic construct
APMFPNQSAGL

SEQ ID NO: 459 - protein, 11 aa, synthetic construct
GSRDQEIETIL

SEQ ID NO: 460 - protein, 11 aa, synthetic construct
RSGSIVANEVY

SEQ ID NO: 461 - protein, 11 aa, synthetic construct
TISKDVHIVLR

SEQ ID NO: 462 - protein, 11 aa, synthetic construct
LTDFLAEDGGT

SEQ ID NO: 463 - protein, 11 aa, synthetic construct
RPSREFGFHQV

SEQ ID NO: 464 - protein, 11 aa, synthetic construct
LSETYSQLPKL

SEQ ID NO: 465 - protein, 11 aa, synthetic construct
ASAKKKNKKGK

SEQ ID NO: 466 - protein, 11 aa, synthetic construct
TQAGVEGSGVI

SEQ ID NO: 467 - protein, 11 aa, synthetic construct
MGIGMAHAGIW

SEQ ID NO: 468 - protein, 11 aa, synthetic construct
MGIGMAHAGIW

SEQ ID NO: 469 - protein, 11 aa, synthetic construct
MGIGMAHAGIW

SEQ ID NO: 470 - protein, 10 aa, synthetic construct
GFMDGFLEEE

SEQ ID NO: 471 - protein, 9 aa, synthetic construct
NPISTGAVF

SEQ ID NO: 472 - protein, 9 aa, synthetic construct
NPISTGAVF

SEQ ID NO: 473 - protein, 11 aa, synthetic construct
SLYSDWTWKGR

SEQ ID NO: 474 - protein, 11 aa, synthetic construct
SGVISAHFNLR

SEQ ID NO: 475 - protein, 11 aa, synthetic construct
KVKESKFTTLL

SEQ ID NO: 476 - protein, 11 aa, synthetic construct
GSTYVSKPVSW

SEQ ID NO: 477 - protein, 11 aa, synthetic construct
NMPGKGIMHVR

SEQ ID NO: 478 - protein, 8 aa, synthetic construct
LTVPSFPL

SEQ ID NO: 479 - protein, 8 aa, synthetic construct
LTVPSFPL

SEQ ID NO: 480 - protein, 11 aa, synthetic construct
EQGTRLPRGSW

SEQ ID NO: 481 - protein, 11 aa, synthetic construct
EQGTRLPRGSW

SEQ ID NO: 482 - protein, 11 aa, synthetic construct
ILSLNVEIRGR

SEQ ID NO: 483 - protein, 11 aa, synthetic construct
HLNFRRPFSDY

SEQ ID NO: 484 - protein, 11 aa, synthetic construct
KYPAEVGGGSL

SEQ ID NO: 485 - protein, 10 aa, synthetic construct
FMDGFLEEEA

SEQ ID NO: 486 - protein, 11 aa, synthetic construct
NLSSFAQWQYR

SEQ ID NO: 487 - protein, 11 aa, synthetic construct
NLSSFAQWQYR

SEQ ID NO: 488 - protein, 11 aa, synthetic construct
NLSSFAQWQYR

SEQ ID NO: 489 - protein, 11 aa, synthetic construct
YTRTHGQALTL

SEQ ID NO: 490 - protein, 11 aa, synthetic construct
YTRTHGQALTL

SEQ ID NO: 491 - protein, 11 aa, synthetic construct
YTRTHGQALTL

SEQ ID NO: 492 - protein, 9 aa, synthetic construct
QTKDNFTDF

SEQ ID NO: 493 - protein, 11 aa, synthetic construct
EENGFSFVLVR

SEQ ID NO: 494 - protein, 11 aa, synthetic construct
LLGNPISTGAV

SEQ ID NO: 495 - protein, 11 aa, synthetic construct
LLGNPISTGAV

SEQ ID NO: 496 - protein, 11 aa, synthetic construct
RIISTTRAGVR

SEQ ID NO: 497 - protein, 11 aa, synthetic construct
NPISTGAVFPN

SEQ ID NO: 498 - protein, 11 aa, synthetic construct
NPISTGAVFPN

SEQ ID NO: 499 - protein, 11 aa, synthetic construct
SIQESTPVDER

SEQ ID NO: 500 - protein, 11 aa, synthetic construct
TVPSFPLLHGL

SEQ ID NO: 501 - protein, 11 aa, synthetic construct
TVPSFPLLHGL

SEQ ID NO: 502 - protein, 11 aa, synthetic construct
IAMMTKAAETM

SEQ ID NO: 503 - protein, 11 aa, synthetic construct
IAMMTKAAETM

SEQ ID NO: 504 - protein, 11 aa, synthetic construct
IAMMTKAAETM

SEQ ID NO: 505 - protein, 11 aa, synthetic construct
IAMMTKAAETM

SEQ ID NO: 506 - protein, 11 aa, synthetic construct
IAMMTKAAETM

SEQ ID NO: 507 - protein, 11 aa, synthetic construct
IAMMTKAAETM

SEQ ID NO: 508 - protein, 11 aa, synthetic construct
VEWVASILIKK

SEQ ID NO: 509 - protein, 10 aa, synthetic construct
FLNEDSPGGS

SEQ ID NO: 510 - protein, 11 aa, synthetic construct
SPGSCVRILTA

SEQ ID NO: 511 - protein, 11 aa, synthetic construct
SPGSCVRILTA

SEQ ID NO: 512 - protein, 11 aa, synthetic construct
GFQGSRAASVF

SEQ ID NO: 513 - protein, 11 aa, synthetic construct
EALRQYSPGGF

SEQ ID NO: 514 - protein, 11 aa, synthetic construct
GPGDGGNKDHW

SEQ ID NO: 515 - protein, 9 aa, synthetic construct
AQEENGFSF

SEQ ID NO: 516 - protein, 11 aa, synthetic construct
ETILANTVKPR

SEQ ID NO: 517 - protein, 11 aa, synthetic construct
AFRTSNSDGSR

SEQ ID NO: 518 - protein, 8 aa, synthetic construct
TTQNGTQF

SEQ ID NO: 519 - protein, 8 aa, synthetic construct
TTQNGTQF

SEQ ID NO: 520 - protein, 8 aa, synthetic construct
TTQNGTQF

SEQ ID NO: 521 - protein, 8 aa, synthetic construct
LVAGEALV

SEQ ID NO: 522 - protein, 8 aa, synthetic construct
LVAGEALV

SEQ ID NO: 523 - protein, 11 aa, synthetic construct
QEIETILANTV

SEQ ID NO: 524 - protein, 9 aa, synthetic construct
FPNRHPTLL

SEQ ID NO: 525 - protein, 9 aa, synthetic construct
FPNRHPTLL

SEQ ID NO: 526 - protein, 11 aa, synthetic construct
ILISEDPFLIT

SEQ ID NO: 527 - protein, 11 aa, synthetic construct
GAVFPNRHPTL

SEQ ID NO: 528 - protein, 11 aa, synthetic construct
GAVFPNRHPTL

SEQ ID NO: 529 - protein, 11 aa, synthetic construct
SREFGFHQVLF

SEQ ID NO: 530 - protein, 10 aa, synthetic construct
AVFPNRHPTL

SEQ ID NO: 531 - protein, 10 aa, synthetic construct
AVFPNRHPTL

SEQ ID NO: 532 - protein, 11 aa, synthetic construct
EAPTLGFMDGF

SEQ ID NO: 533 - protein, 11 aa, synthetic construct
KTRQLQNCERR

SEQ ID NO: 534 - protein, 11 aa, synthetic construct
KTRQLQNCERR

SEQ ID NO: 535 - protein, 8 aa, synthetic construct
YRKYPAEV

SEQ ID NO: 536 - protein, 11 aa, synthetic construct
LAWKSHILLAK

SEQ ID NO: 537 - protein, 11 aa, synthetic construct
LAWKSHILLAK

SEQ ID NO: 538 - protein, 11 aa, synthetic construct
SEAQEENGFSF

SEQ ID NO: 539 - protein, 11 aa, synthetic construct
NSRPQVIRQPR

SEQ ID NO: 540 - protein, 11 aa, synthetic construct
QFPPLGMKDKV

SEQ ID NO: 541 - protein, 9 aa, synthetic construct
AETMIEAMI

SEQ ID NO: 542 - protein, 9 aa, synthetic construct
AETMIEAMI

SEQ ID NO: 543 - protein, 9 aa, synthetic construct
AETMIEAMI

SEQ ID NO: 544 - protein, 9 aa, synthetic construct
AETMIEAMI

SEQ ID NO: 545 - protein, 9 aa, synthetic construct
AETMIEAMI

SEQ ID NO: 546 - protein, 9 aa, synthetic construct
AETMIEAMI

SEQ ID NO: 547 - protein, 9 aa, synthetic construct
AETMIEAMI

SEQ ID NO: 548 - protein, 9 aa, synthetic construct
AETMIEAMI

SEQ ID NO: 549 - protein, 11 aa, synthetic construct
KSAPATRPASK

SEQ ID NO: 550 - protein, 11 aa, synthetic construct
KSAPATRPASK

SEQ ID NO: 551 - protein, 11 aa, synthetic construct
NLLLSHPEGHL

SEQ ID NO: 552 - protein, 11 aa, synthetic construct
FPPLGMKDKVL

SEQ ID NO: 553 - protein, 11 aa, synthetic construct
TTEEAGTAMKT

SEQ ID NO: 554 - protein, 11 aa, synthetic construct
TTEEAGTAMKT

SEQ ID NO: 555 - protein, 11 aa, synthetic construct
VEGSGVISAHF

SEQ ID NO: 556 - protein, 9 aa, synthetic construct
ILIKKGTDL

SEQ ID NO: 557 - protein, 11 aa, synthetic construct
HHTTQNGTQFR

SEQ ID NO: 558 - protein, 11 aa, synthetic construct
HHTTQNGTQFR

SEQ ID NO: 559 - protein, 11 aa, synthetic construct
HHTTQNGTQFR

SEQ ID NO: 560 - protein, 11 aa, synthetic construct
SETYSQLPKLK

SEQ ID NO: 561 - protein, 11 aa, synthetic construct
LNFSKRENAFR

SEQ ID NO: 562 - protein, 11 aa, synthetic construct
QFSEAQEENGF

SEQ ID NO: 563 - protein, 11 aa, synthetic construct
ANHKATTNSRR

SEQ ID NO: 564 - protein, 11 aa, synthetic construct
ANHKATTNSRR

SEQ ID NO: 565 - protein, 11 aa, synthetic construct
DQDSRSAPEPK

SEQ ID NO: 566 - protein, 11 aa, synthetic construct
VFPNRHPTLLF

SEQ ID NO: 567 - protein, 11 aa, synthetic construct
VFPNRHPTLLF

SEQ ID NO: 568 - protein, 10 aa, synthetic construct
GQYGETLSLL

SEQ ID NO: 569 - protein, 11 aa, synthetic construct
LRSQDAGHSKK

SEQ ID NO: 570 - protein, 11 aa, synthetic construct
ETYSQLPKLKM

SEQ ID NO: 571 - protein, 10 aa, synthetic construct
YPAEVGGGSL

SEQ ID NO: 572 - protein, 10 aa, synthetic construct
RQYSPGGFQG

SEQ ID NO: 573 - protein, 11 aa, synthetic construct
RFKRMKSVEVR

SEQ ID NO: 574 - protein, 9 aa, synthetic construct
HTTQNGTQF

SEQ ID NO: 575 - protein, 9 aa, synthetic construct
HTTQNGTQF

SEQ ID NO: 576 - protein, 9 aa, synthetic construct
HTTQNGTQF

SEQ ID NO: 577 - protein, 11 aa, synthetic construct
SWSTEGRDAHK

SEQ ID NO: 578 - protein, 11 aa, synthetic construct
SWSTEGRDAHK

SEQ ID NO: 579 - protein, 8 aa, synthetic construct
LVEEAPMF

SEQ ID NO: 580 - protein, 11 aa, synthetic construct
WADETMTWKEM

SEQ ID NO: 581 - protein, 11 aa, synthetic construct
FLAEDGGTGGG

SEQ ID NO: 582 - protein, 11 aa, synthetic construct
HWRAGQTKDNF

SEQ ID NO: 583 - protein, 8 aa, synthetic construct
NGFSFVLV

SEQ ID NO: 584 - protein, 11 aa, synthetic construct
TLRLSETYSQL

SEQ ID NO: 585 - protein, 11 aa, synthetic construct
NLETLRLSETY

SEQ ID NO: 586 - protein, 11 aa, synthetic construct
MQKMEATGRGW

SEQ ID NO: 587 - protein, 9 aa, synthetic construct
IQTGIGMGI

SEQ ID NO: 588 - protein, 9 aa, synthetic construct
IQTGIGMGI

SEQ ID NO: 589 - protein, 11 aa, synthetic construct
SPWGGRGGRIT

SEQ ID NO: 590 - protein, 11 aa, synthetic construct
SQAKTAVGQSF

SEQ ID NO: 591 - protein, 11 aa, synthetic construct
TESQFPPLGMK

SEQ ID NO: 592 - protein, 11 aa, synthetic construct
SVNMPGKGIMH

SEQ ID NO: 593 - protein, 11 aa, synthetic construct
KKPPMQMGLKY

SEQ ID NO: 594 - protein, 11 aa, synthetic construct
HHPKAMASSVF

SEQ ID NO: 595 - protein, 11 aa, synthetic construct
TDTPKENAMWR

SEQ ID NO: 596 - protein, 11 aa, synthetic construct
TDTPKENAMWR

SEQ ID NO: 597 - protein, 10 aa, synthetic construct
QYSPGGFQGS

SEQ ID NO: 598 - protein, 11 aa, synthetic construct
LEYECWPEIRY

SEQ ID NO: 599 - protein, 11 aa, synthetic construct
FHHTPQKESTL

SEQ ID NO: 600 - protein, 11 aa, synthetic construct
FHHTPQKESTL

SEQ ID NO: 601 - protein, 11 aa, synthetic construct
FHHTPQKESTL

SEQ ID NO: 602 - protein, 11 aa, synthetic construct
PKAMASSVFPK

SEQ ID NO: 603 - protein, 9 aa, synthetic construct
SEDPFLITI

SEQ ID NO: 604 - protein, 11 aa, synthetic construct
MFPNQSAGLMK

SEQ ID NO: 605 - protein, 11 aa, synthetic construct
EVGGGSLEAWK

SEQ ID NO: 606 - protein, 9 aa, synthetic construct
EEEGNVEWV

SEQ ID NO: 607 - protein, 9 aa, synthetic construct
LETSIGIVM

SEQ ID NO: 608 - protein, 11 aa, synthetic construct
TLKGHSDKGHL

SEQ ID NO: 609 - protein, 11 aa, synthetic construct
TLKGHSDKGHL

SEQ ID NO: 610 - protein, 11 aa, synthetic construct
QEENGFSFVLV

SEQ ID NO: 611 - protein, 11 aa, synthetic construct
TVIGLGKAEEK